European Patent Application EP 4 342 490 A1, published March 27, 2024. Title: nucleic acid lipid nanoparticle vaccine for influenza. Applicant: DAIICHI SANKYO COMPANY, LIMITED. The sequence listing filed with the application follows.

SEQUENCE LISTING (58 sequences)

SEQ ID NO: 1 - DNA, 1930 bp, Artificial Sequence
  template DNA
gctagcgtaatacgactcactatagggagacccaagctacatttgcttctgacacaactgtgttcactagcaacctcaaacagacaccgccaccatgaaggccaacctgctggtgctgctgtgtgctctggctgccgctgatgccgataccatctgtatcggctaccacgccaacaacagcaccgacaccgtggataccgtgctggaaaagaacgtgaccgtgacacacagcgtgaacctgctcgaggacagccacaatggcaagctgtgccggctgaagggaattgcccctctgcagctgggcaagtgcaatatcgctggatggctgctgggcaaccccgagtgtgatcctctgctgcctgtcagatcctggtcctacatcgtggaaacccctaacagcgagaacggcatctgctaccccggcgacttcatcgactacgaggaactgagagaacagctgagcagcgtgtccagcttcgagagattcgagatcttccccaaagagagcagctggcccaaccacaacaccaatggcgtgacagccgcctgttctcacgagggcaagagcagcttctaccggaacctgctgtggctgaccgagaaagagggcagctaccccaagctgaagaactcctacgtgaacaagaaaggcaaagaggtgctggtcctctggggcatccaccatcctccaaacagcaaagagcagcagaacctgtaccagaacgagaatgcctacgtgtccgtggtcaccagcaactacaaccggcggttcacacctgagatcgccgagaggcctaaagtgcgcgatcaggccggcagaatgaactactactggaccctgctgaagcccggcgacaccatcatctttgaggccaacggcaacctgatcgcccctatgtacgccttcgctctgagcagaggctttggcagcggcatcatcacctccaacgccagcatgcacgagtgcaacaccaagtgtcagacacccctgggcgctatcaacagcagcctgccttaccagaacattcaccccgtgaccatcggcgagtgccccaaatacgtcagatccgccaagctgagaatggtcaccggcctgagaaacatccccagcatccagtccagaggcctgtttggcgccattgccggctttatcgaaggcggctggaccggcatgatcgacggatggtacggataccaccaccagaatgagcaaggcagcggctacgccgccgatcagaaaagcacacagaacgccatcaacggcatcaccaacaaagtgaacaccgtgatcgagaagatgaacatccagttcaccgccgtgggcaaagagttcaacaagctggaaaaacggatggaaaacctcaacaagaaggtggacgacggcttcctggacatctggacctacaatgccgagctgctcgtgctcctggaaaacgagagaaccctggacttccacgacagcaacgtgaagaatctgtacgagaaagtgaagtcccagctcaagaacaacgccaaagagatcggcaacggctgcttcgagttctaccacaagtgcgacaacgagtgcatggaaagcgtgcggaacggcacctacgactaccctaagtacagcgaggaaagcaagctgaaccgcgaaaaagtggacggcgtgaagctggaatccatgggcatctaccagattctggccatctacagcaccgtggcctctagcctggtgcttctggtttctctgggcgccatcagcttttggatgtgcagcaatggcagcctgcagtgccggatctgcatctgagctcgctttcttgctgtccaatttctattaaaggttcctttgttccctaagtccaactactaaactgggggatattatgaagggccttgagcatctggattctgcctaataaaaaacatttattttcattgcgaattc

SEQ ID NO: 2 - RNA, 1905 nt, Artificial Sequence
  A/Puerto Rico/8/34(subtype H1) mRNA-001
gggagacccaagcuacauuugcuucugacacaacuguguucacuagcaaccucaaacagacaccgccaccaugaaggccaaccugcuggugcugcugugugcucuggcugccgcugaugccgauaccaucuguaucggcuaccacgccaacaacagcaccgacaccguggauaccgugcuggaaaagaacgugaccgugacacacagcgugaaccugcucgaggacagccacaauggcaagcugugccggcugaagggaauugccccucugcagcugggcaagugcaauaucgcuggauggcugcugggcaaccccgagugugauccucugcugccugucagauccugguccuacaucguggaaaccccuaacagcgagaacggcaucugcuaccccggcgacuucaucgacuacgaggaacugagagaacagcugagcagcguguccagcuucgagagauucgagaucuuccccaaagagagcagcuggcccaaccacaacaccaauggcgugacagccgccuguucucacgagggcaagagcagcuucuaccggaaccugcuguggcugaccgagaaagagggcagcuaccccaagcugaagaacuccuacgugaacaagaaaggcaaagaggugcugguccucuggggcauccaccauccuccaaacagcaaagagcagcagaaccuguaccagaacgagaaugccuacguguccguggucaccagcaacuacaaccggcgguucacaccugagaucgccgagaggccuaaagugcgcgaucaggccggcagaaugaacuacuacuggacccugcugaagcccggcgacaccaucaucuuugaggccaacggcaaccugaucgccccuauguacgccuucgcucugagcagaggcuuuggcagcggcaucaucaccuccaacgccagcaugcacgagugcaacaccaagugucagacaccccugggcgcuaucaacagcagccugccuuaccagaacauucaccccgugaccaucggcgagugccccaaauacgucagauccgccaagcugagaauggucaccggccugagaaacauccccagcauccaguccagaggccuguuuggcgccauugccggcuuuaucgaaggcggcuggaccggcaugaucgacggaugguacggauaccaccaccagaaugagcaaggcagcggcuacgccgccgaucagaaaagcacacagaacgccaucaacggcaucaccaacaaagugaacaccgugaucgagaagaugaacauccaguucaccgccgugggcaaagaguucaacaagcuggaaaaacggauggaaaaccucaacaagaagguggacgacggcuuccuggacaucuggaccuacaaugccgagcugcucgugcuccuggaaaacgagagaacccuggacuuccacgacagcaacgugaagaaucuguacgagaaagugaagucccagcucaagaacaacgccaaagagaucggcaacggcugcuucgaguucuaccacaagugcgacaacgagugcauggaaagcgugcggaacggcaccuacgacuacccuaaguacagcgaggaaagcaagcugaaccgcgaaaaaguggacggcgugaagcuggaauccaugggcaucuaccagauucuggccaucuacagcaccguggccucuagccuggugcuucugguuucucugggcgccaucagcuuuuggaugugcagcaauggcagccugcagugccggaucugcaucugagcucgcuuucuugcuguccaauuucuauuaaagguuccuuuguucccuaaguccaacuacuaaacugggggauauuaugaagggccuugagcaucuggauucugccuaauaaaaaacauuuauuuucauugcgaauu

SEQ ID NO: 3 - DNA, 2036 bp, Artificial Sequence
  DNA fragment
gctagcgtaatacgactcactatagggagacccaagctacatttgcttctgacacaactgtgttcactagcaacctcaaacagacaccgccaccatgaaggccaacctgctggtgctgctgtgtgctctggctgccgctgatgccgataccatctgtatcggctaccacgccaacaacagcaccgacaccgtggataccgtgctggaaaagaacgtgaccgtgacacacagcgtgaacctgctcgaggacagccacaatggcaagctgtgccggctgaagggaattgcccctctgcagctgggcaagtgcaatatcgctggatggctgctgggcaaccccgagtgtgatcctctgctgcctgtcagatcctggtcctacatcgtggaaacccctaacagcgagaacggcatctgctaccccggcgacttcatcgactacgaggaactgagagaacagctgagcagcgtgtccagcttcgagagattcgagatcttccccaaagagagcagctggcccaaccacaacaccaatggcgtgacagccgcctgttctcacgagggcaagagcagcttctaccggaacctgctgtggctgaccgagaaagagggcagctaccccaagctgaagaactcctacgtgaacaagaaaggcaaagaggtgctggtcctctggggcatccaccatcctccaaacagcaaagagcagcagaacctgtaccagaacgagaatgcctacgtgtccgtggtcaccagcaactacaaccggcggttcacacctgagatcgccgagaggcctaaagtgcgcgatcaggccggcagaatgaactactactggaccctgctgaagcccggcgacaccatcatctttgaggccaacggcaacctgatcgcccctatgtacgccttcgctctgagcagaggctttggcagcggcatcatcacctccaacgccagcatgcacgagtgcaacaccaagtgtcagacacccctgggcgctatcaacagcagcctgccttaccagaacattcaccccgtgaccatcggcgagtgccccaaatacgtcagatccgccaagctgagaatggtcaccggcctgagaaacatccccagcatccagtccagaggcctgtttggcgccattgccggctttatcgaaggcggctggaccggcatgatcgacggatggtacggataccaccaccagaatgagcaaggcagcggctacgccgccgatcagaaaagcacacagaacgccatcaacggcatcaccaacaaagtgaacaccgtgatcgagaagatgaacatccagttcaccgccgtgggcaaagagttcaacaagctggaaaaacggatggaaaacctcaacaagaaggtggacgacggcttcctggacatctggacctacaatgccgagctgctcgtgctcctggaaaacgagagaaccctggacttccacgacagcaacgtgaagaatctgtacgagaaagtgaagtcccagctcaagaacaacgccaaagagatcggcaacggctgcttcgagttctaccacaagtgcgacaacgagtgcatggaaagcgtgcggaacggcacctacgactaccctaagtacagcgaggaaagcaagctgaaccgcgaaaaagtggacggcgtgaagctggaatccatgggcatctaccagattctggccatctacagcaccgtggcctctagcctggtgcttctggtttctctgggcgccatcagcttttggatgtgcagcaatggcagcctgcagtgccggatctgcatctgagctcgctttcttgctgtccaatttctattaaaggttcctttgttccctaagtccaactactaaactgggggatattatgaagggccttgagcatctggattctgcctaataaaaaacatttattttcattgcaaaaaaaaaaaaaaaaaaaaaaaaaaaaaaaaaaaaaaaaaaaaaaaaaaaaaaaaaaaaaaaaaaaaaaaaaaaaaaaaaaaaaaaaaaaaaaaaaaaaaagagcactagt

SEQ ID NO: 4 - DNA, 24 bp, Artificial Sequence
  sense primer
taatacgactcactataaggagac

SEQ ID NO: 5 - DNA, 129 bp, Artificial Sequence
  antisense primer
ttttttttttttttttttttttttttttttttttttttttttttttttttttttttttttttttttttttttttttttttttttttttttttttttttttgcaatgaaaataaatgttttttattaggc

SEQ ID NO: 6 - DNA, 2017 bp, Artificial Sequence
  template DNA
taatacgactcactataaggagacccaagctacatttgcttctgacacaactgtgttcactagcaacctcaaacagacaccgccaccatgaaggccaacctgctggtgctgctgtgtgctctggctgccgctgatgccgataccatctgtatcggctaccacgccaacaacagcaccgacaccgtggataccgtgctggaaaagaacgtgaccgtgacacacagcgtgaacctgctcgaggacagccacaatggcaagctgtgccggctgaagggaattgcccctctgcagctgggcaagtgcaatatcgctggatggctgctgggcaaccccgagtgtgatcctctgctgcctgtcagatcctggtcctacatcgtggaaacccctaacagcgagaacggcatctgctaccccggcgacttcatcgactacgaggaactgagagaacagctgagcagcgtgtccagcttcgagagattcgagatcttccccaaagagagcagctggcccaaccacaacaccaatggcgtgacagccgcctgttctcacgagggcaagagcagcttctaccggaacctgctgtggctgaccgagaaagagggcagctaccccaagctgaagaactcctacgtgaacaagaaaggcaaagaggtgctggtcctctggggcatccaccatcctccaaacagcaaagagcagcagaacctgtaccagaacgagaatgcctacgtgtccgtggtcaccagcaactacaaccggcggttcacacctgagatcgccgagaggcctaaagtgcgcgatcaggccggcagaatgaactactactggaccctgctgaagcccggcgacaccatcatctttgaggccaacggcaacctgatcgcccctatgtacgccttcgctctgagcagaggctttggcagcggcatcatcacctccaacgccagcatgcacgagtgcaacaccaagtgtcagacacccctgggcgctatcaacagcagcctgccttaccagaacattcaccccgtgaccatcggcgagtgccccaaatacgtcagatccgccaagctgagaatggtcaccggcctgagaaacatccccagcatccagtccagaggcctgtttggcgccattgccggctttatcgaaggcggctggaccggcatgatcgacggatggtacggataccaccaccagaatgagcaaggcagcggctacgccgccgatcagaaaagcacacagaacgccatcaacggcatcaccaacaaagtgaacaccgtgatcgagaagatgaacatccagttcaccgccgtgggcaaagagttcaacaagctggaaaaacggatggaaaacctcaacaagaaggtggacgacggcttcctggacatctggacctacaatgccgagctgctcgtgctcctggaaaacgagagaaccctggacttccacgacagcaacgtgaagaatctgtacgagaaagtgaagtcccagctcaagaacaacgccaaagagatcggcaacggctgcttcgagttctaccacaagtgcgacaacgagtgcatggaaagcgtgcggaacggcacctacgactaccctaagtacagcgaggaaagcaagctgaaccgcgaaaaagtggacggcgtgaagctggaatccatgggcatctaccagattctggccatctacagcaccgtggcctctagcctggtgcttctggtttctctgggcgccatcagcttttggatgtgcagcaatggcagcctgcagtgccggatctgcatctgagctcgctttcttgctgtccaatttctattaaaggttcctttgttccctaagtccaactactaaactgggggatattatgaagggccttgagcatctggattctgcctaataaaaaacatttattttcattgcaaaaaaaaaaaaaaaaaaaaaaaaaaaaaaaaaaaaaaaaaaaaaaaaaaaaaaaaaaaaaaaaaaaaaaaaaaaaaaaaaaaaaaaaaaaaaaaaaaaa

SEQ ID NO: 7 - RNA, 2000 nt, Artificial Sequence
  A/Puerto Rico/8/34 (subtype H1) HA mRNA-002 or 003
aggagacccaagcuacauuugcuucugacacaacuguguucacuagcaaccucaaacagacaccgccaccaugaaggccaaccugcuggugcugcugugugcucuggcugccgcugaugccgauaccaucuguaucggcuaccacgccaacaacagcaccgacaccguggauaccgugcuggaaaagaacgugaccgugacacacagcgugaaccugcucgaggacagccacaauggcaagcugugccggcugaagggaauugccccucugcagcugggcaagugcaauaucgcuggauggcugcugggcaaccccgagugugauccucugcugccugucagauccugguccuacaucguggaaaccccuaacagcgagaacggcaucugcuaccccggcgacuucaucgacuacgaggaacugagagaacagcugagcagcguguccagcuucgagagauucgagaucuuccccaaagagagcagcuggcccaaccacaacaccaauggcgugacagccgccuguucucacgagggcaagagcagcuucuaccggaaccugcuguggcugaccgagaaagagggcagcuaccccaagcugaagaacuccuacgugaacaagaaaggcaaagaggugcugguccucuggggcauccaccauccuccaaacagcaaagagcagcagaaccuguaccagaacgagaaugccuacguguccguggucaccagcaacuacaaccggcgguucacaccugagaucgccgagaggccuaaagugcgcgaucaggccggcagaaugaacuacuacuggacccugcugaagcccggcgacaccaucaucuuugaggccaacggcaaccugaucgccccuauguacgccuucgcucugagcagaggcuuuggcagcggcaucaucaccuccaacgccagcaugcacgagugcaacaccaagugucagacaccccugggcgcuaucaacagcagccugccuuaccagaacauucaccccgugaccaucggcgagugccccaaauacgucagauccgccaagcugagaauggucaccggccugagaaacauccccagcauccaguccagaggccuguuuggcgccauugccggcuuuaucgaaggcggcuggaccggcaugaucgacggaugguacggauaccaccaccagaaugagcaaggcagcggcuacgccgccgaucagaaaagcacacagaacgccaucaacggcaucaccaacaaagugaacaccgugaucgagaagaugaacauccaguucaccgccgugggcaaagaguucaacaagcuggaaaaacggauggaaaaccucaacaagaagguggacgacggcuuccuggacaucuggaccuacaaugccgagcugcucgugcuccuggaaaacgagagaacccuggacuuccacgacagcaacgugaagaaucuguacgagaaagugaagucccagcucaagaacaacgccaaagagaucggcaacggcugcuucgaguucuaccacaagugcgacaacgagugcauggaaagcgugcggaacggcaccuacgacuacccuaaguacagcgaggaaagcaagcugaaccgcgaaaaaguggacggcgugaagcuggaauccaugggcaucuaccagauucuggccaucuacagcaccguggccucuagccuggugcuucugguuucucugggcgccaucagcuuuuggaugugcagcaauggcagccugcagugccggaucugcaucugagcucgcuuucuugcuguccaauuucuauuaaagguuccuuuguucccuaaguccaacuacuaaacugggggauauuaugaagggccuugagcaucuggauucugccuaauaaaaaacauuuauuuucauugcaaaaaaaaaaaaaaaaaaaaaaaaaaaaaaaaaaaaaaaaaaaaaaaaaaaaaaaaaaaaaaaaaaaaaaaaaaaaaaaaaaaaaaaaaaaaaaaaaaaa

SEQ ID NO: 8 - DNA, 2039 bp, Artificial Sequence
  DNA fragment
gctagcgtaatacgactcactataaggagacccaagctacatttgcttctgacacaactgtgttcactagcaacctcaaacagacaccgccaccatgaaggccatcctggtggtgctgctgtacaccttcaccaccgccaacgccgacacactgtgtatcggctaccacgccaacaacagcaccgacaccgtggataccgtgctggaaaagaacgtgaccgtgacacacagcgtgaacctgctggaagataagcacaacggcaagctgtgcaagctgagaggcgtggcacctctgcacctgggcaagtgtaatatcgccggctggatcctgggcaaccctgagtgtgaaagcctgagcacagccagcagctggtcctacatcgtggaaaccagcaacagcgacaacggcacatgctaccccggcgacttcatcaactacgaggaactgcgggaacagctgagcagcgtgtccagcttcgagagattcgagatcttccccaaggcctccagctggcccaaccacgattctaacaaaggcgtgaccgccgcctgtcctcatgccggcgctaagagcttctacaagaacctgatctggctggtcaagaagggcaacagctaccccaagctgaaccagagctacatcaacgacaagggcaaagaggtgctggtcctctggggcatccaccatcctagcacaacagccgatcagcagagcctgtaccagaacgccgatgcctatgtgttcgtgggcaccagccggtacagcaagaagttcaagcccgagatcgccaccagacctaaagtgcgggatcaagaggcccggatgaactactactggaccctggtggaacccggcgacaagatcacatttgaggccaccggcaacctggtggtccccagatacgccttcaccatggaaagaaatgccggcagcggcatcatcatcagcgacacccctgtgcacgactgcaacaccacctgtcagacacctgagggcgccatcaataccagcctgcctttccagaacattcaccccatcaccatcggcaagtgccccaaatacgtgaagtccaccaagctgaggctggccacaggcctgagaaatgtgccctccatccagagcagaggcctgtttggagccattgccggctttatcgaaggcggctggacaggcatggtggacggatggtacggataccaccaccagaacgagcaaggctctggctatgccgccgacctgaagtctacccagaatgccatcgataagatcaccaacaaagtgaacagcgtgatcgagaagatgaacacccagttcaccgccgtgggaaaagagttcaaccacctggaaaagcgcatcgagaacctgaacaagaaggtggacgacggcttcctggacatctggacctacaatgccgagctgctggtgctcctggaaaacgagagaaccctggactaccacgacagcaacgtgaagaacctgtacgagaaagtgcgcaaccagctgaagaacaacgccaaagagatcggcaacggctgcttcgagttctaccacaagtgcgacaatacctgcatggaaagcgtgaagaatggcacctacgactaccctaagtacagcgaggaagccaaactgaaccgcgagaagatcgacggcgtgaagctggaaagcacccggatctatcagatcctggccatctacagcaccgtggccagttctctggtgctggtggtttctctgggcgctatcagcttctggatgtgcagcaatggcagcctgcagtgccggatctgcatctgagctcgctttcttgctgtccaatttctattaaaggttcctttgttccctaagtccaactactaaactgggggatattatgaagggccttgagcatctggattctgcctaataaaaaacatttattttcattgcaaaaaaaaaaaaaaaaaaaaaaaaaaaaaaaaaaaaaaaaaaaaaaaaaaaaaaaaaaaaaaaaaaaaaaaaaaaaaaaaaaaaaaaaaaaaaaaaaaaaaagagcactagt

SEQ ID NO: 9 - DNA, 2020 bp, Artificial Sequence
  template DNA
taatacgactcactataaggagacccaagctacatttgcttctgacacaactgtgttcactagcaacctcaaacagacaccgccaccatgaaggccatcctggtggtgctgctgtacaccttcaccaccgccaacgccgacacactgtgtatcggctaccacgccaacaacagcaccgacaccgtggataccgtgctggaaaagaacgtgaccgtgacacacagcgtgaacctgctggaagataagcacaacggcaagctgtgcaagctgagaggcgtggcacctctgcacctgggcaagtgtaatatcgccggctggatcctgggcaaccctgagtgtgaaagcctgagcacagccagcagctggtcctacatcgtggaaaccagcaacagcgacaacggcacatgctaccccggcgacttcatcaactacgaggaactgcgggaacagctgagcagcgtgtccagcttcgagagattcgagatcttccccaaggcctccagctggcccaaccacgattctaacaaaggcgtgaccgccgcctgtcctcatgccggcgctaagagcttctacaagaacctgatctggctggtcaagaagggcaacagctaccccaagctgaaccagagctacatcaacgacaagggcaaagaggtgctggtcctctggggcatccaccatcctagcacaacagccgatcagcagagcctgtaccagaacgccgatgcctatgtgttcgtgggcaccagccggtacagcaagaagttcaagcccgagatcgccaccagacctaaagtgcgggatcaagaggcccggatgaactactactggaccctggtggaacccggcgacaagatcacatttgaggccaccggcaacctggtggtccccagatacgccttcaccatggaaagaaatgccggcagcggcatcatcatcagcgacacccctgtgcacgactgcaacaccacctgtcagacacctgagggcgccatcaataccagcctgcctttccagaacattcaccccatcaccatcggcaagtgccccaaatacgtgaagtccaccaagctgaggctggccacaggcctgagaaatgtgccctccatccagagcagaggcctgtttggagccattgccggctttatcgaaggcggctggacaggcatggtggacggatggtacggataccaccaccagaacgagcaaggctctggctatgccgccgacctgaagtctacccagaatgccatcgataagatcaccaacaaagtgaacagcgtgatcgagaagatgaacacccagttcaccgccgtgggaaaagagttcaaccacctggaaaagcgcatcgagaacctgaacaagaaggtggacgacggcttcctggacatctggacctacaatgccgagctgctggtgctcctggaaaacgagagaaccctggactaccacgacagcaacgtgaagaacctgtacgagaaagtgcgcaaccagctgaagaacaacgccaaagagatcggcaacggctgcttcgagttctaccacaagtgcgacaatacctgcatggaaagcgtgaagaatggcacctacgactaccctaagtacagcgaggaagccaaactgaaccgcgagaagatcgacggcgtgaagctggaaagcacccggatctatcagatcctggccatctacagcaccgtggccagttctctggtgctggtggtttctctgggcgctatcagcttctggatgtgcagcaatggcagcctgcagtgccggatctgcatctgagctcgctttcttgctgtccaatttctattaaaggttcctttgttccctaagtccaactactaaactgggggatattatgaagggccttgagcatctggattctgcctaataaaaaacatttattttcattgcaaaaaaaaaaaaaaaaaaaaaaaaaaaaaaaaaaaaaaaaaaaaaaaaaaaaaaaaaaaaaaaaaaaaaaaaaaaaaaaaaaaaaaaaaaaaaaaaaaaa

SEQ ID NO: 10 - RNA, 2003 nt, Artificial Sequence
  A/Singapore/GP1908/2015 (subtype H1) HA mRNA-001, 002 or 003
aggagacccaagcuacauuugcuucugacacaacuguguucacuagcaaccucaaacagacaccgccaccaugaaggccauccugguggugcugcuguacaccuucaccaccgccaacgccgacacacuguguaucggcuaccacgccaacaacagcaccgacaccguggauaccgugcuggaaaagaacgugaccgugacacacagcgugaaccugcuggaagauaagcacaacggcaagcugugcaagcugagaggcguggcaccucugcaccugggcaaguguaauaucgccggcuggauccugggcaacccugagugugaaagccugagcacagccagcagcugguccuacaucguggaaaccagcaacagcgacaacggcacaugcuaccccggcgacuucaucaacuacgaggaacugcgggaacagcugagcagcguguccagcuucgagagauucgagaucuuccccaaggccuccagcuggcccaaccacgauucuaacaaaggcgugaccgccgccuguccucaugccggcgcuaagagcuucuacaagaaccugaucuggcuggucaagaagggcaacagcuaccccaagcugaaccagagcuacaucaacgacaagggcaaagaggugcugguccucuggggcauccaccauccuagcacaacagccgaucagcagagccuguaccagaacgccgaugccuauguguucgugggcaccagccgguacagcaagaaguucaagcccgagaucgccaccagaccuaaagugcgggaucaagaggcccggaugaacuacuacuggacccugguggaacccggcgacaagaucacauuugaggccaccggcaaccuggugguccccagauacgccuucaccauggaaagaaaugccggcagcggcaucaucaucagcgacaccccugugcacgacugcaacaccaccugucagacaccugagggcgccaucaauaccagccugccuuuccagaacauucaccccaucaccaucggcaagugccccaaauacgugaaguccaccaagcugaggcuggccacaggccugagaaaugugcccuccauccagagcagaggccuguuuggagccauugccggcuuuaucgaaggcggcuggacaggcaugguggacggaugguacggauaccaccaccagaacgagcaaggcucuggcuaugccgccgaccugaagucuacccagaaugccaucgauaagaucaccaacaaagugaacagcgugaucgagaagaugaacacccaguucaccgccgugggaaaagaguucaaccaccuggaaaagcgcaucgagaaccugaacaagaagguggacgacggcuuccuggacaucuggaccuacaaugccgagcugcuggugcuccuggaaaacgagagaacccuggacuaccacgacagcaacgugaagaaccuguacgagaaagugcgcaaccagcugaagaacaacgccaaagagaucggcaacggcugcuucgaguucuaccacaagugcgacaauaccugcauggaaagcgugaagaauggcaccuacgacuacccuaaguacagcgaggaagccaaacugaaccgcgagaagaucgacggcgugaagcuggaaagcacccggaucuaucagauccuggccaucuacagcaccguggccaguucucuggugcuggugguuucucugggcgcuaucagcuucuggaugugcagcaauggcagccugcagugccggaucugcaucugagcucgcuuucuugcuguccaauuucuauuaaagguuccuuuguucccuaaguccaacuacuaaacugggggauauuaugaagggccuugagcaucuggauucugccuaauaaaaaacauuuauuuucauugcaaaaaaaaaaaaaaaaaaaaaaaaaaaaaaaaaaaaaaaaaaaaaaaaaaaaaaaaaaaaaaaaaaaaaaaaaaaaaaaaaaaaaaaaaaaaaaaaaaaa

SEQ ID NO: 11 - DNA, 2039 bp, Artificial Sequence
  DNA fragment
gctagcgtaatacgactcactataaggagacccaagctacatttgcttctgacacaactgtgttcactagcaacctcaaacagacaccgccaccatgaagaccatcattgccctgagctacatcctgtgcctggtgttcgcccagaagatccccggcaacgacaatagcaccgccacactgtgtctgggccatcacgctgtgcctaacggcaccatcgtgaaaaccatcaccaacgaccggatcgaagtgaccaacgccacagagctggtgcagaacagcagcatcggcgagatctgcgatagccctcaccagatcctggacggcgagaactgcacactgatcgatgccctgctgggcgatcctcagtgtgacggcttccagaacaagaaatgggacctgttcgtggaacggtccaaggcctacagcaactgctacccctacgacgtgccagactacgccagcctgagatctctggtggcctctagcggcaccctggaattcaagaacgagagcttcaactggaccggcgtgacccagaatggcacaagcagcgcctgtatcagaggcagcagctccagcttcttcagcagactgaactggctgacccacctgaactacaagtaccccgctctgaacgtgaccatgcctaacaaagagcagttcgacaagctgtacatctggggcgtgcaccatcctggcaccgacaaggatcagatcttcccatacgctcagagcagcggcagaatcaccgtgtccaccaagagaagccagcaggccgtgattcccaacatcggcagcagacctagaatccggggcatccccagccggatcagcatctactggacaatcgtgaagcccggcgacatcctgctgatcaacagcaccggcaatctgatcgcccctcggggctacttcaagatcagaagcggcaagagcagcatcatgcggagcgacgcccctatcggcaagtgcaagagcgagtgcatcaccccaaacggcagcatccccaacgacaagcccttccagaatgtgaaccggatcacctacggcgcctgtcctagatacgtgaagcacagcaccctgaagctggccaccggcatgagaaatgtgcccgagaagcagaccagaggcatcttcggagccattgccggcttcatcgagaacggctgggaaggcatggtggacggatggtacggcttcagacaccagaacagcgaaggcagaggacaggccgctgacctgaaatctacacaggccgccatcgaccagatcaacggcaagctgaaccggctgatcggcaagaccaacgagaagttccaccagatcgagaaagagttcagcgaggtcgagggcagagtgcaggacctcgagaaatacgtggaagataccaagatcgacctgtggtcctacaatgccgagctgctggtggccctggaaaaccagcacaccatcgacctgaccgacagcgagatgaacaagctgttcgaaaagaccaagaagcagctgcgcgagaacgccgaggatatgggcaacggctgctttaagatctaccacaagtgcgacaacgcctgcatcgagagcatccggaacgagacatacgaccacaacgtgtacagagatgaggccctgaacaaccggttccagatcaaaggcgtggaactgaagtccggctacaaggactggatcctgtggatcagcttcgccatcagctgctttctgctgtgcgtggcactgctgggcttcatcatgtgggcctgccagaaaggcaacatccggtgcaacatctgcatctgagctcgctttcttgctgtccaatttctattaaaggttcctttgttccctaagtccaactactaaactgggggatattatgaagggccttgagcatctggattctgcctaataaaaaacatttattttcattgcaaaaaaaaaaaaaaaaaaaaaaaaaaaaaaaaaaaaaaaaaaaaaaaaaaaaaaaaaaaaaaaaaaaaaaaaaaaaaaaaaaaaaaaaaaaaaaaaaaaaaagagcactagt

SEQ ID NO: 12 - DNA, 2020 bp, Artificial Sequence
  template DNA
taatacgactcactataaggagacccaagctacatttgcttctgacacaactgtgttcactagcaacctcaaacagacaccgccaccatgaagaccatcattgccctgagctacatcctgtgcctggtgttcgcccagaagatccccggcaacgacaatagcaccgccacactgtgtctgggccatcacgctgtgcctaacggcaccatcgtgaaaaccatcaccaacgaccggatcgaagtgaccaacgccacagagctggtgcagaacagcagcatcggcgagatctgcgatagccctcaccagatcctggacggcgagaactgcacactgatcgatgccctgctgggcgatcctcagtgtgacggcttccagaacaagaaatgggacctgttcgtggaacggtccaaggcctacagcaactgctacccctacgacgtgccagactacgccagcctgagatctctggtggcctctagcggcaccctggaattcaagaacgagagcttcaactggaccggcgtgacccagaatggcacaagcagcgcctgtatcagaggcagcagctccagcttcttcagcagactgaactggctgacccacctgaactacaagtaccccgctctgaacgtgaccatgcctaacaaagagcagttcgacaagctgtacatctggggcgtgcaccatcctggcaccgacaaggatcagatcttcccatacgctcagagcagcggcagaatcaccgtgtccaccaagagaagccagcaggccgtgattcccaacatcggcagcagacctagaatccggggcatccccagccggatcagcatctactggacaatcgtgaagcccggcgacatcctgctgatcaacagcaccggcaatctgatcgcccctcggggctacttcaagatcagaagcggcaagagcagcatcatgcggagcgacgcccctatcggcaagtgcaagagcgagtgcatcaccccaaacggcagcatccccaacgacaagcccttccagaatgtgaaccggatcacctacggcgcctgtcctagatacgtgaagcacagcaccctgaagctggccaccggcatgagaaatgtgcccgagaagcagaccagaggcatcttcggagccattgccggcttcatcgagaacggctgggaaggcatggtggacggatggtacggcttcagacaccagaacagcgaaggcagaggacaggccgctgacctgaaatctacacaggccgccatcgaccagatcaacggcaagctgaaccggctgatcggcaagaccaacgagaagttccaccagatcgagaaagagttcagcgaggtcgagggcagagtgcaggacctcgagaaatacgtggaagataccaagatcgacctgtggtcctacaatgccgagctgctggtggccctggaaaaccagcacaccatcgacctgaccgacagcgagatgaacaagctgttcgaaaagaccaagaagcagctgcgcgagaacgccgaggatatgggcaacggctgctttaagatctaccacaagtgcgacaacgcctgcatcgagagcatccggaacgagacatacgaccacaacgtgtacagagatgaggccctgaacaaccggttccagatcaaaggcgtggaactgaagtccggctacaaggactggatcctgtggatcagcttcgccatcagctgctttctgctgtgcgtggcactgctgggcttcatcatgtgggcctgccagaaaggcaacatccggtgcaacatctgcatctgagctcgctttcttgctgtccaatttctattaaaggttcctttgttccctaagtccaactactaaactgggggatattatgaagggccttgagcatctggattctgcctaataaaaaacatttattttcattgcaaaaaaaaaaaaaaaaaaaaaaaaaaaaaaaaaaaaaaaaaaaaaaaaaaaaaaaaaaaaaaaaaaaaaaaaaaaaaaaaaaaaaaaaaaaaaaaaaaaa

SEQ ID NO: 13 - RNA, 2003 nt, Artificial Sequence
  A/Singapore/INFIMH-16-0019/2016 (subtype H3) HA mRNA-001 or 002
aggagacccaagcuacauuugcuucugacacaacuguguucacuagcaaccucaaacagacaccgccaccaugaagaccaucauugcccugagcuacauccugugccugguguucgcccagaagauccccggcaacgacaauagcaccgccacacugugucugggccaucacgcugugccuaacggcaccaucgugaaaaccaucaccaacgaccggaucgaagugaccaacgccacagagcuggugcagaacagcagcaucggcgagaucugcgauagcccucaccagauccuggacggcgagaacugcacacugaucgaugcccugcugggcgauccucagugugacggcuuccagaacaagaaaugggaccuguucguggaacgguccaaggccuacagcaacugcuaccccuacgacgugccagacuacgccagccugagaucucugguggccucuagcggcacccuggaauucaagaacgagagcuucaacuggaccggcgugacccagaauggcacaagcagcgccuguaucagaggcagcagcuccagcuucuucagcagacugaacuggcugacccaccugaacuacaaguaccccgcucugaacgugaccaugccuaacaaagagcaguucgacaagcuguacaucuggggcgugcaccauccuggcaccgacaaggaucagaucuucccauacgcucagagcagcggcagaaucaccguguccaccaagagaagccagcaggccgugauucccaacaucggcagcagaccuagaauccggggcauccccagccggaucagcaucuacuggacaaucgugaagcccggcgacauccugcugaucaacagcaccggcaaucugaucgccccucggggcuacuucaagaucagaagcggcaagagcagcaucaugcggagcgacgccccuaucggcaagugcaagagcgagugcaucaccccaaacggcagcauccccaacgacaagcccuuccagaaugugaaccggaucaccuacggcgccuguccuagauacgugaagcacagcacccugaagcuggccaccggcaugagaaaugugcccgagaagcagaccagaggcaucuucggagccauugccggcuucaucgagaacggcugggaaggcaugguggacggaugguacggcuucagacaccagaacagcgaaggcagaggacaggccgcugaccugaaaucuacacaggccgccaucgaccagaucaacggcaagcugaaccggcugaucggcaagaccaacgagaaguuccaccagaucgagaaagaguucagcgaggucgagggcagagugcaggaccucgagaaauacguggaagauaccaagaucgaccugugguccuacaaugccgagcugcugguggcccuggaaaaccagcacaccaucgaccugaccgacagcgagaugaacaagcuguucgaaaagaccaagaagcagcugcgcgagaacgccgaggauaugggcaacggcugcuuuaagaucuaccacaagugcgacaacgccugcaucgagagcauccggaacgagacauacgaccacaacguguacagagaugaggcccugaacaaccgguuccagaucaaaggcguggaacugaaguccggcuacaaggacuggauccuguggaucagcuucgccaucagcugcuuucugcugugcguggcacugcugggcuucaucaugugggccugccagaaaggcaacauccggugcaacaucugcaucugagcucgcuuucuugcuguccaauuucuauuaaagguuccuuuguucccuaaguccaacuacuaaacugggggauauuaugaagggccuugagcaucuggauucugccuaauaaaaaacauuuauuuucauugcaaaaaaaaaaaaaaaaaaaaaaaaaaaaaaaaaaaaaaaaaaaaaaaaaaaaaaaaaaaaaaaaaaaaaaaaaaaaaaaaaaaaaaaaaaaaaaaaaaaa

SEQ ID NO: 14 - DNA, 2093 bp, Artificial Sequence
  DNA fragment
gctagcgtaatacgactcactataaggagacccaagctacatttgcttctgacacaactgtgttcactagcaacctcaaacagacaccgccaccatgaaggccatcatcgtgctgctgatggtggtcaccagcaacgccgacagaatctgcaccggcatcaccagcagcaacagccctcacgtggtcaagacagccacacagggcgaagtgaatgtgaccggcgtgatccctctgaccaccacacctaccaagagctacttcgccaacctgaagggcaccagaaccagaggcaagctgtgccccgattgcctgaactgcaccgatctggatgtggccctgggcagacctatgtgcgtgggaacaacacctagcgccaaggccagcatcctgcatgaagtgcggcctgtgaccagcggctgcttccctattatgcacgaccggaccaagatcagacagctgcccaatctgctgcggggctacgagaagatcaggctgagcacccagaacgtgatcgacgccgaaaaagctcctggcggcccttacagactgggcacatctggctcttgccccaacgctacaagcaagatcggcttcttcgccaccatggcctgggccgtgcctaaggacaactacaagaacgccaccaatcctctgaccgtggaagtgccctacatctgtaccgaaggcgaggaccagatcaccgtgtggggctttcacagcgacgacaagacccagatgaagtccctgtacggcgacagcaaccctcagaagtttaccagcagcgccaacggcgtgaccacacactatgtgtcccagatcggcgacttccccgaccagacagaagatggcggactgcctcagagcggcagaatcgtggtggactacatgatgcagaagcccggcaagaccggcaccatcgtgtatcagagaggcgtcctgctgccacagaaagtttggtgcgccagcggccggtccaaagtgatcaaaggatccctgcctctgatcggcgaggccgactgtctgcacgaagaatatggcggcctgaacaagagcaagccctactacacaggcaagcacgccaaagccatcggcaactgccctatctgggtcaagacccctctgaagctggccaacggcaccaagtatagacctccagccaagctgctgaaagagcggggcttctttggagctatcgccggctttcttgaaggcggctgggagggaatgattgccggctggcatggctacacatctcatggcgcacatggcgtggcagtggccgctgatctgaagtctacacaagaggccatcaacaagatcaccaagaacctgaacagcctgagcgagctggaagtgaagaacctgcagagactgtccggcgccatggacgagctgcacaacgagatcctggaactggacgagaaggtggacgacctgagagccgataccatctccagccagattgagctggcagtgctgctgtccaacgagggcatcatcaacagcgaggacgagcatctgctggccctggaacggaagctgaagaagatgctgggacccagcgccgtggatatcggcaatggctgcttcgagacaaagcacaagtgcaaccagacctgcctggacagaattgccgccggaacctttaacgccggcgagtttagcctgcctaccttcgacagcctgaacatcacagccgccagcctgaatgacgacggcctggacaatcacaccatcctgctgtactactccaccgccgcctcttctctggccgtgacactgatgctggctatcttcatcgtgtacatggtgtccagagacaacgtgtcctgcagcatctgtctctgagctcgctttcttgctgtccaatttctattaaaggttcctttgttccctaagtccaactactaaactgggggatattatgaagggccttgagcatctggattctgcctaataaaaaacatttattttcattgcaaaaaaaaaaaaaaaaaaaaaaaaaaaaaaaaaaaaaaaaaaaaaaaaaaaaaaaaaaaaaaaaaaaaaaaaaaaaaaaaaaaaaaaaaaaaaaaaaaaaaagagcactagt

SEQ ID NO: 15 - DNA, 2074 bp, Artificial Sequence
  template DNA
taatacgactcactataaggagacccaagctacatttgcttctgacacaactgtgttcactagcaacctcaaacagacaccgccaccatgaaggccatcatcgtgctgctgatggtggtcaccagcaacgccgacagaatctgcaccggcatcaccagcagcaacagccctcacgtggtcaagacagccacacagggcgaagtgaatgtgaccggcgtgatccctctgaccaccacacctaccaagagctacttcgccaacctgaagggcaccagaaccagaggcaagctgtgccccgattgcctgaactgcaccgatctggatgtggccctgggcagacctatgtgcgtgggaacaacacctagcgccaaggccagcatcctgcatgaagtgcggcctgtgaccagcggctgcttccctattatgcacgaccggaccaagatcagacagctgcccaatctgctgcggggctacgagaagatcaggctgagcacccagaacgtgatcgacgccgaaaaagctcctggcggcccttacagactgggcacatctggctcttgccccaacgctacaagcaagatcggcttcttcgccaccatggcctgggccgtgcctaaggacaactacaagaacgccaccaatcctctgaccgtggaagtgccctacatctgtaccgaaggcgaggaccagatcaccgtgtggggctttcacagcgacgacaagacccagatgaagtccctgtacggcgacagcaaccctcagaagtttaccagcagcgccaacggcgtgaccacacactatgtgtcccagatcggcgacttccccgaccagacagaagatggcggactgcctcagagcggcagaatcgtggtggactacatgatgcagaagcccggcaagaccggcaccatcgtgtatcagagaggcgtcctgctgccacagaaagtttggtgcgccagcggccggtccaaagtgatcaaaggatccctgcctctgatcggcgaggccgactgtctgcacgaagaatatggcggcctgaacaagagcaagccctactacacaggcaagcacgccaaagccatcggcaactgccctatctgggtcaagacccctctgaagctggccaacggcaccaagtatagacctccagccaagctgctgaaagagcggggcttctttggagctatcgccggctttcttgaaggcggctgggagggaatgattgccggctggcatggctacacatctcatggcgcacatggcgtggcagtggccgctgatctgaagtctacacaagaggccatcaacaagatcaccaagaacctgaacagcctgagcgagctggaagtgaagaacctgcagagactgtccggcgccatggacgagctgcacaacgagatcctggaactggacgagaaggtggacgacctgagagccgataccatctccagccagattgagctggcagtgctgctgtccaacgagggcatcatcaacagcgaggacgagcatctgctggccctggaacggaagctgaagaagatgctgggacccagcgccgtggatatcggcaatggctgcttcgagacaaagcacaagtgcaaccagacctgcctggacagaattgccgccggaacctttaacgccggcgagtttagcctgcctaccttcgacagcctgaacatcacagccgccagcctgaatgacgacggcctggacaatcacaccatcctgctgtactactccaccgccgcctcttctctggccgtgacactgatgctggctatcttcatcgtgtacatggtgtccagagacaacgtgtcctgcagcatctgtctctgagctcgctttcttgctgtccaatttctattaaaggttcctttgttccctaagtccaactactaaactgggggatattatgaagggccttgagcatctggattctgcctaataaaaaacatttattttcattgcaaaaaaaaaaaaaaaaaaaaaaaaaaaaaaaaaaaaaaaaaaaaaaaaaaaaaaaaaaaaaaaaaaaaaaaaaaaaaaaaaaaaaaaaaaaaaaaaaaaa

SEQ ID NO: 16 - RNA, 2057 nt, Artificial Sequence
  B/Phuket/3073/2013 (yamagata lineage) HA mRNA-001 or 002
aggagacccaagcuacauuugcuucugacacaacuguguucacuagcaaccucaaacagacaccgccaccaugaaggccaucaucgugcugcugaugguggucaccagcaacgccgacagaaucugcaccggcaucaccagcagcaacagcccucacguggucaagacagccacacagggcgaagugaaugugaccggcgugaucccucugaccaccacaccuaccaagagcuacuucgccaaccugaagggcaccagaaccagaggcaagcugugccccgauugccugaacugcaccgaucuggauguggcccugggcagaccuaugugcgugggaacaacaccuagcgccaaggccagcauccugcaugaagugcggccugugaccagcggcugcuucccuauuaugcacgaccggaccaagaucagacagcugcccaaucugcugcggggcuacgagaagaucaggcugagcacccagaacgugaucgacgccgaaaaagcuccuggcggcccuuacagacugggcacaucuggcucuugccccaacgcuacaagcaagaucggcuucuucgccaccauggccugggccgugccuaaggacaacuacaagaacgccaccaauccucugaccguggaagugcccuacaucuguaccgaaggcgaggaccagaucaccguguggggcuuucacagcgacgacaagacccagaugaagucccuguacggcgacagcaacccucagaaguuuaccagcagcgccaacggcgugaccacacacuaugugucccagaucggcgacuuccccgaccagacagaagauggcggacugccucagagcggcagaaucgugguggacuacaugaugcagaagcccggcaagaccggcaccaucguguaucagagaggcguccugcugccacagaaaguuuggugcgccagcggccgguccaaagugaucaaaggaucccugccucugaucggcgaggccgacugucugcacgaagaauauggcggccugaacaagagcaagcccuacuacacaggcaagcacgccaaagccaucggcaacugcccuaucugggucaagaccccucugaagcuggccaacggcaccaaguauagaccuccagccaagcugcugaaagagcggggcuucuuuggagcuaucgccggcuuucuugaaggcggcugggagggaaugauugccggcuggcauggcuacacaucucauggcgcacauggcguggcaguggccgcugaucugaagucuacacaagaggccaucaacaagaucaccaagaaccugaacagccugagcgagcuggaagugaagaaccugcagagacuguccggcgccauggacgagcugcacaacgagauccuggaacuggacgagaagguggacgaccugagagccgauaccaucuccagccagauugagcuggcagugcugcuguccaacgagggcaucaucaacagcgaggacgagcaucugcuggcccuggaacggaagcugaagaagaugcugggacccagcgccguggauaucggcaauggcugcuucgagacaaagcacaagugcaaccagaccugccuggacagaauugccgccggaaccuuuaacgccggcgaguuuagccugccuaccuucgacagccugaacaucacagccgccagccugaaugacgacggccuggacaaucacaccauccugcuguacuacuccaccgccgccucuucucuggccgugacacugaugcuggcuaucuucaucguguacaugguguccagagacaacguguccugcagcaucugucucugagcucgcuuucuugcuguccaauuucuauuaaagguuccuuuguucccuaaguccaacuacuaaacugggggauauuaugaagggccuugagcaucuggauucugccuaauaaaaaacauuuauuuucauugcaaaaaaaaaaaaaaaaaaaaaaaaaaaaaaaaaaaaaaaaaaaaaaaaaaaaaaaaaaaaaaaaaaaaaaaaaaaaaaaaaaaaaaaaaaaaaaaaaaaa

SEQ ID NO: 17 - DNA, 2090 bp, Artificial Sequence
  DNA fragment
gctagcgtaatacgactcactataaggagacccaagctacatttgcttctgacacaactgtgttcactagcaacctcaaacagacaccgccaccatgaaggccatcatcgtgctgctgatggtggtcaccagcaacgccgacagaatctgcaccggcatcaccagcagcaacagccctcacgtggtcaagacagccacacagggcgaagtgaatgtgaccggcgtgatccctctgaccaccacacctaccaagagccacttcgccaacctgaagggcaccgagacaagaggcaagctgtgccccaagtgcctgaactgcaccgatctggatgtggccctgggcagacctaagtgtaccggcaagatccctagcgccagagtgtccatcctgcacgaagtgcggcctgtgaccagcggctgctttcccattatgcacgaccggaccaagatcagacagctgcccaatctgctgcggggctatgaacatgtgcggctgagcacccacaacgtgatcaacgccgaagatgctcctggcggcccttacaagatcggcacatctggctcttgccccaacattaccaacggcaacggcttcttcgccaccatggcttgggctgtgcccgacaagaacaagaccgccaccaatccactgaccatcgaggtgccctacgtgtgcacagaaggcgaggatcagatcaccgtgtggggcttccacagcgacaacgagatccagatggccaagctgtacggcgacagcaagccccagaagtttaccagctctgccaacggcgtgaccacacactacgtgtcccagatcggcggcttccccaatcagacagaagatggcggactgccccagagcggaagaatcgtggtggactacatggtgcagaagtccggcaagaccggcacaatcacataccagcggggaatcctgctgcctcagaaagtttggtgcgccagcggccggtccaaagtgatcaaaggatccctgcctctgatcggcgaggccgattgtctgcacgagaaatacggcggcctgaacaagagcaagccctactacacaggcgagcacgccaaggccatcggcaactgtcctatctgggtcaagacccctctgaagctggccaacggcaccaagtatagacctccagccaagctgctgaaagagcggggcttctttggagctatcgccggctttcttgaaggcggctgggagggaatgattgccggctggcatggctacacatctcatggcgcacatggcgtggcagtggccgctgatctgaagtctacacaagaggccatcaacaagatcaccaagaacctgaacagcctgagcgagctggaagtgaagaacctgcagagactgtccggcgccatggacgagctgcacaatgagatcctggaactggacgagaaggtggacgacctgagagccgataccatctccagccagattgagctggcagtgctgctgtccaacgagggcatcatcaacagcgaggacgagcatctgctggccctggaacggaagctgaagaagatgctgggcccaagcgccgtggaaatcggcaatggctgcttcgagacaaagcacaagtgcaaccagacctgcctggacaagattgccgccggaacatttgacgccggcgagtttagcctgcctaccttcgacagcctgaacatcacagccgccagcctgaatgacgacggcctggataatcacaccatcctgctgtactactccaccgccgcctcttctctggccgtgacactgatgatcgccatctttgtggtgtacatggtgtccagagacaacgtgtcctgcagcatctgtctctgagctcgctttcttgctgtccaatttctattaaaggttcctttgttccctaagtccaactactaaactgggggatattatgaagggccttgagcatctggattctgcctaataaaaaacatttattttcattgcaaaaaaaaaaaaaaaaaaaaaaaaaaaaaaaaaaaaaaaaaaaaaaaaaaaaaaaaaaaaaaaaaaaaaaaaaaaaaaaaaaaaaaaaaaaaaaaaaaaaaagagcactagt

SEQ ID NO: 18 - DNA, 2071 bp, Artificial Sequence
  template DNA
taatacgactcactataaggagacccaagctacatttgcttctgacacaactgtgttcactagcaacctcaaacagacaccgccaccatgaaggccatcatcgtgctgctgatggtggtcaccagcaacgccgacagaatctgcaccggcatcaccagcagcaacagccctcacgtggtcaagacagccacacagggcgaagtgaatgtgaccggcgtgatccctctgaccaccacacctaccaagagccacttcgccaacctgaagggcaccgagacaagaggcaagctgtgccccaagtgcctgaactgcaccgatctggatgtggccctgggcagacctaagtgtaccggcaagatccctagcgccagagtgtccatcctgcacgaagtgcggcctgtgaccagcggctgctttcccattatgcacgaccggaccaagatcagacagctgcccaatctgctgcggggctatgaacatgtgcggctgagcacccacaacgtgatcaacgccgaagatgctcctggcggcccttacaagatcggcacatctggctcttgccccaacattaccaacggcaacggcttcttcgccaccatggcttgggctgtgcccgacaagaacaagaccgccaccaatccactgaccatcgaggtgccctacgtgtgcacagaaggcgaggatcagatcaccgtgtggggcttccacagcgacaacgagatccagatggccaagctgtacggcgacagcaagccccagaagtttaccagctctgccaacggcgtgaccacacactacgtgtcccagatcggcggcttccccaatcagacagaagatggcggactgccccagagcggaagaatcgtggtggactacatggtgcagaagtccggcaagaccggcacaatcacataccagcggggaatcctgctgcctcagaaagtttggtgcgccagcggccggtccaaagtgatcaaaggatccctgcctctgatcggcgaggccgattgtctgcacgagaaatacggcggcctgaacaagagcaagccctactacacaggcgagcacgccaaggccatcggcaactgtcctatctgggtcaagacccctctgaagctggccaacggcaccaagtatagacctccagccaagctgctgaaagagcggggcttctttggagctatcgccggctttcttgaaggcggctgggagggaatgattgccggctggcatggctacacatctcatggcgcacatggcgtggcagtggccgctgatctgaagtctacacaagaggccatcaacaagatcaccaagaacctgaacagcctgagcgagctggaagtgaagaacctgcagagactgtccggcgccatggacgagctgcacaatgagatcctggaactggacgagaaggtggacgacctgagagccgataccatctccagccagattgagctggcagtgctgctgtccaacgagggcatcatcaacagcgaggacgagcatctgctggccctggaacggaagctgaagaagatgctgggcccaagcgccgtggaaatcggcaatggctgcttcgagacaaagcacaagtgcaaccagacctgcctggacaagattgccgccggaacatttgacgccggcgagtttagcctgcctaccttcgacagcctgaacatcacagccgccagcctgaatgacgacggcctggataatcacaccatcctgctgtactactccaccgccgcctcttctctggccgtgacactgatgatcgccatctttgtggtgtacatggtgtccagagacaacgtgtcctgcagcatctgtctctgagctcgctttcttgctgtccaatttctattaaaggttcctttgttccctaagtccaactactaaactgggggatattatgaagggccttgagcatctggattctgcctaataaaaaacatttattttcattgcaaaaaaaaaaaaaaaaaaaaaaaaaaaaaaaaaaaaaaaaaaaaaaaaaaaaaaaaaaaaaaaaaaaaaaaaaaaaaaaaaaaaaaaaaaaaaaaaaaaa

SEQ ID NO: 19 - RNA, 2054 nt, Artificial Sequence
  B/Maryland/15/2016 (Victoria lineage) HA mRNA-001 or 002
aggagacccaagcuacauuugcuucugacacaacuguguucacuagcaaccucaaacagacaccgccaccaugaaggccaucaucgugcugcugaugguggucaccagcaacgccgacagaaucugcaccggcaucaccagcagcaacagcccucacguggucaagacagccacacagggcgaagugaaugugaccggcgugaucccucugaccaccacaccuaccaagagccacuucgccaaccugaagggcaccgagacaagaggcaagcugugccccaagugccugaacugcaccgaucuggauguggcccugggcagaccuaaguguaccggcaagaucccuagcgccagaguguccauccugcacgaagugcggccugugaccagcggcugcuuucccauuaugcacgaccggaccaagaucagacagcugcccaaucugcugcggggcuaugaacaugugcggcugagcacccacaacgugaucaacgccgaagaugcuccuggcggcccuuacaagaucggcacaucuggcucuugccccaacauuaccaacggcaacggcuucuucgccaccauggcuugggcugugcccgacaagaacaagaccgccaccaauccacugaccaucgaggugcccuacgugugcacagaaggcgaggaucagaucaccguguggggcuuccacagcgacaacgagauccagauggccaagcuguacggcgacagcaagccccagaaguuuaccagcucugccaacggcgugaccacacacuacgugucccagaucggcggcuuccccaaucagacagaagauggcggacugccccagagcggaagaaucgugguggacuacauggugcagaaguccggcaagaccggcacaaucacauaccagcggggaauccugcugccucagaaaguuuggugcgccagcggccgguccaaagugaucaaaggaucccugccucugaucggcgaggccgauugucugcacgagaaauacggcggccugaacaagagcaagcccuacuacacaggcgagcacgccaaggccaucggcaacuguccuaucugggucaagaccccucugaagcuggccaacggcaccaaguauagaccuccagccaagcugcugaaagagcggggcuucuuuggagcuaucgccggcuuucuugaaggcggcugggagggaaugauugccggcuggcauggcuacacaucucauggcgcacauggcguggcaguggccgcugaucugaagucuacacaagaggccaucaacaagaucaccaagaaccugaacagccugagcgagcuggaagugaagaaccugcagagacuguccggcgccauggacgagcugcacaaugagauccuggaacuggacgagaagguggacgaccugagagccgauaccaucuccagccagauugagcuggcagugcugcuguccaacgagggcaucaucaacagcgaggacgagcaucugcuggcccuggaacggaagcugaagaagaugcugggcccaagcgccguggaaaucggcaauggcugcuucgagacaaagcacaagugcaaccagaccugccuggacaagauugccgccggaacauuugacgccggcgaguuuagccugccuaccuucgacagccugaacaucacagccgccagccugaaugacgacggccuggauaaucacaccauccugcuguacuacuccaccgccgccucuucucuggccgugacacugaugaucgccaucuuugugguguacaugguguccagagacaacguguccugcagcaucugucucugagcucgcuuucuugcuguccaauuucuauuaaagguuccuuuguucccuaaguccaacuacuaaacugggggauauuaugaagggccuugagcaucuggauucugccuaauaaaaaacauuuauuuucauugcaaaaaaaaaaaaaaaaaaaaaaaaaaaaaaaaaaaaaaaaaaaaaaaaaaaaaaaaaaaaaaaaaaaaaaaaaaaaaaaaaaaaaaaaaaaaaaaaaaaa

SEQ ID NO: 20 - protein, 565 aa, Influenza A virus
MKANLLVLLCALAAADADTICIGYHANNSTDTVDTVLEKNVTVTHSVNLLEDSHNGKLCRLKGIAPLQLGKCNIAGWLLGNPECDPLLPVRSWSYIVETPNSENGICYPGDFIDYEELREQLSSVSSFERFEIFPKESSWPNHNTNGVTAACSHEGKSSFYRNLLWLTEKEGSYPKLKNSYVNKKGKEVLVLWGIHHPPNSKEQQNLYQNENAYVSVVTSNYNRRFTPEIAERPKVRDQAGRMNYYWTLLKPGDTIIFEANGNLIAPMYAFALSRGFGSGIITSNASMHECNTKCQTPLGAINSSLPYQNIHPVTIGECPKYVRSAKLRMVTGLRNIPSIQSRGLFGAIAGFIEGGWTGMIDGWYGYHHQNEQGSGYAADQKSTQNAINGITNKVNTVIEKMNIQFTAVGKEFNKLEKRMENLNKKVDDGFLDIWTYNAELLVLLENERTLDFHDSNVKNLYEKVKSQLKNNAKEIGNGCFEFYHKCDNECMESVRNGTYDYPKYSEESKLNREKVDGVKLESMGIYQILAIYSTVASSLVLLVSLGAISFWMCSNGSLQCRICI

SEQ ID NO: 21 - protein, 566 aa, Influenza A virus
MKAILVVLLYTFTTANADTLCIGYHANNSTDTVDTVLEKNVTVTHSVNLLEDKHNGKLCKLRGVAPLHLGKCNIAGWILGNPECESLSTASSWSYIVETSNSDNGTCYPGDFINYEELREQLSSVSSFERFEIFPKASSWPNHDSNKGVTAACPHAGAKSFYKNLIWLVKKGNSYPKLNQSYINDKGKEVLVLWGIHHPSTTADQQSLYQNADAYVFVGTSRYSKKFKPEIATRPKVRDQEARMNYYWTLVEPGDKITFEATGNLVVPRYAFTMERNAGSGIIISDTPVHDCNTTCQTPEGAINTSLPFQNIHPITIGKCPKYVKSTKLRLATGLRNVPSIQSRGLFGAIAGFIEGGWTGMVDGWYGYHHQNEQGSGYAADLKSTQNAIDKITNKVNSVIEKMNTQFTAVGKEFNHLEKRIENLNKKVDDGFLDIWTYNAELLVLLENERTLDYHDSNVKNLYEKVRNQLKNNAKEIGNGCFEFYHKCDNTCMESVKNGTYDYPKYSEEAKLNREKIDGVKLESTRIYQILAIYSTVASSLVLVVSLGAISFWMCSNGSLQCRICI

SEQ ID NO: 22 - protein, 566 aa, Influenza A virus
MKTIIALSYILCLVFAQKIPGNDNSTATLCLGHHAVPNGTIVKTITNDRIEVTNATELVQNSSIGEICDSPHQILDGENCTLIDALLGDPQCDGFQNKKWDLFVERSKAYSNCYPYDVPDYASLRSLVASSGTLEFKNESFNWTGVTQNGTSSACIRGSSSSFFSRLNWLTHLNYKYPALNVTMPNKEQFDKLYIWGVHHPGTDKDQIFPYAQSSGRITVSTKRSQQAVIPNIGSRPRIRGIPSRISIYWTIVKPGDILLINSTGNLIAPRGYFKIRSGKSSIMRSDAPIGKCKSECITPNGSIPNDKPFQNVNRITYGACPRYVKHSTLKLATGMRNVPEKQTRGIFGAIAGFIENGWEGMVDGWYGFRHQNSEGRGQAADLKSTQAAIDQINGKLNRLIGKTNEKFHQIEKEFSEVEGRVQDLEKYVEDTKIDLWSYNAELLVALENQHTIDLTDSEMNKLFEKTKKQLRENAEDMGNGCFKIYHKCDNACIESIRNETYDHNVYRDEALNNRFQIKGVELKSGYKDWILWISFAISCFLLCVALLGFIMWACQKGNIRCNICI

SEQ ID NO: 23 - protein, 584 aa, Influenza B virus
MKAIIVLLMVVTSNADRICTGITSSNSPHVVKTATQGEVNVTGVIPLTTTPTKSYFANLKGTRTRGKLCPDCLNCTDLDVALGRPMCVGTTPSAKASILHEVRPVTSGCFPIMHDRTKIRQLPNLLRGYEKIRLSTQNVIDAEKAPGGPYRLGTSGSCPNATSKIGFFATMAWAVPKDNYKNATNPLTVEVPYICTEGEDQITVWGFHSDDKTQMKSLYGDSNPQKFTSSANGVTTHYVSQIGDFPDQTEDGGLPQSGRIVVDYMMQKPGKTGTIVYQRGVLLPQKVWCASGRSKVIKGSLPLIGEADCLHEEYGGLNKSKPYYTGKHAKAIGNCPIWVKTPLKLANGTKYRPPAKLLKERGFFGAIAGFLEGGWEGMIAGWHGYTSHGAHGVAVAADLKSTQEAINKITKNLNSLSELEVKNLQRLSGAMDELHNEILELDEKVDDLRADTISSQIELAVLLSNEGIINSEDEHLLALERKLKKMLGPSAVDIGNGCFETKHKCNQTCLDRIAAGTFNAGEFSLPTFDSLNITAASLNDDGLDNHTILLYYSTAASSLAVTLMLAIFIVYMVSRDNVSCSICL

SEQ ID NO: 24 - protein, 583 aa, Influenza B virus
MKAIIVLLMVVTSNADRICTGITSSNSPHVVKTATQGEVNVTGVIPLTTTPTKSHFANLKGTETRGKLCPKCLNCTDLDVALGRPKCTGKIPSARVSILHEVRPVTSGCFPIMHDRTKIRQLPNLLRGYEHVRLSTHNVINAEDAPGGPYKIGTSGSCPNITNGNGFFATMAWAVPDKNKTATNPLTIEVPYVCTEGEDQITVWGFHSDNEIQMAKLYGDSKPQKFTSSANGVTTHYVSQIGGFPNQTEDGGLPQSGRIVVDYMVQKSGKTGTITYQRGILLPQKVWCASGRSKVIKGSLPLIGEADCLHEKYGGLNKSKPYYTGEHAKAIGNCPIWVKTPLKLANGTKYRPPAKLLKERGFFGAIAGFLEGGWEGMIAGWHGYTSHGAHGVAVAADLKSTQEAINKITKNLNSLSELEVKNLQRLSGAMDELHNEILELDEKVDDLRADTISSQIELAVLLSNEGIINSEDEHLLALERKLKKMLGPSAVEIGNGCFETKHKCNQTCLDKIAAGTFDAGEFSLPTFDSLNITAASLNDDGLDNHTILLYYSTAASSLAVTLMIAIFVVYMVSRDNVSCSICL

SEQ ID NO: 25 - protein, 7 aa, Artificial Sequence
  proteolytic cleavage site
RGRKRRS

SEQ ID NO: 26 - DNA, 2045 bp, Artificial Sequence
  template DNA sequence for A/Guangdong-Maonan/SWL1536/2019 polyA110
gctagcgtaatacgactcactataaggagacccaagctacatttgcttctgacacaactgtgttcactagcaacctcaaacagacaccgccaccatgaaggccatcctggtggtgctgctgtacaccttcaccaccgccaacgccgacacactgtgcatcggctaccacgccaacaacagcaccgacaccgtggacaccgtgctggaaaagaacgtgaccgtgacacacagcgtgaacctgctggaagacaagcacaacggcaagctgtgcaagctgagaggcgtggcacccctgcacctgggcaagtgcaacatcgccggctggatcctgggcaaccccgagtgcgaaagcctgagcaccgccagaagctggagctacatcgtggaaaccagcaacagcgacaacggcacatgctaccccggcgacttcatcaactacgaggaactgcgggaacagctgagcagcgtgagcagcttcgagagattcgagatcttccccaagaccagcagctggcccaaccacgacagcgacaaaggcgtgacagccgcctgcccccacgccggcgccaagagcttctacaagaacctgatctggctggtcaagaagggcaacagctaccccaagctgaaccagacctacatcaacgacaagggcaaagaggtgctggtcctctggggcatccaccaccccccaacaatcgccgcccaagagagcctgtaccagaacgccgacgcctacgtgttcgtgggcaccagcagatacagcaagaagttcaagcccgagatcgccaccaggcccaaagtgcgggaccaagagggcagaatgaactactactggaccctggtggaacccggcgacaagatcacattcgaggccaccggcaacctggtggtccccagatacgccttcaccatggaaagagacgccggcagcggcatcatcatcagcgacacccccgtgcacgactgcaacaccacctgccagacacccgagggcgccatcaacaccagcctgcccttccagaacgtgcaccccatcaccatcggcaagtgccccaaatacgtgaagtccaccaagctgaggctggccacaggcctgagaaacgtgcccagcatccagagcagaggcctgttcggagccatcgccggcttcatcgaaggcggctggacaggcatggtggacggatggtacggataccaccaccagaacgagcaaggcagcggctacgccgccgacctgaagtccacccagaacgccatcgacaagatcaccaacaaagtgaacagcgtgatcgagaagatgaacacccagttcaccgccgtgggaaaagagttcaaccacctggaaaagcgcatcgagaacctgaacaagaaggtggacgacggcttcctggacatctggacctacaacgccgagctgctcgtgctgctcgagaacgagagaaccctggactaccacgacagcaacgtgaagaacctgtacgagaaagtgcgcaaccagctgaagaacaacgccaaagagatcggcaacggctgcttcgagttctaccacaagtgcgacaacacctgcatggaaagcgtgaagaacggcacctacgactaccccaagtacagcgaggaagccaaactgaaccgcgagaagatcgacggcgtgaagctggaaagcacccggatctaccagatcctggccatctacagcaccgtggccagcagcctggtgctggtggtgagcctgggcgccatcagcttctggatgtgcagcaacggcagcctgcagtgccggatctgcatctgagctcgctttcttgctgtccaatttctattaaaggttcctttgttccctaagtccaactactaaactgggggatattatgaagggccttgagcatctggattctgcctaataaaaaacatttattttcattgcaaaaaaaaaaaaaaaaaaaaaaaaaaaaaaaaaaaaaaaaaaaaaaaaaaaaaaaaaaaaaaaaaaaaaaaaaaaaaaaaaaaaaaaaaaaaaaaaaaaaaaaaaaaaaacgaagagc

SEQ ID NO: 27 - DNA, 2030 bp, Artificial Sequence
  template DNA sequence for A/Guangdong-Maonan/SWL1536/2019 polyA95
gctagcgtaatacgactcactataaggagacccaagctacatttgcttctgacacaactgtgttcactagcaacctcaaacagacaccgccaccatgaaggccatcctggtggtgctgctgtacaccttcaccaccgccaacgccgacacactgtgcatcggctaccacgccaacaacagcaccgacaccgtggacaccgtgctggaaaagaacgtgaccgtgacacacagcgtgaacctgctggaagacaagcacaacggcaagctgtgcaagctgagaggcgtggcacccctgcacctgggcaagtgcaacatcgccggctggatcctgggcaaccccgagtgcgaaagcctgagcaccgccagaagctggagctacatcgtggaaaccagcaacagcgacaacggcacatgctaccccggcgacttcatcaactacgaggaactgcgggaacagctgagcagcgtgagcagcttcgagagattcgagatcttccccaagaccagcagctggcccaaccacgacagcgacaaaggcgtgacagccgcctgcccccacgccggcgccaagagcttctacaagaacctgatctggctggtcaagaagggcaacagctaccccaagctgaaccagacctacatcaacgacaagggcaaagaggtgctggtcctctggggcatccaccaccccccaacaatcgccgcccaagagagcctgtaccagaacgccgacgcctacgtgttcgtgggcaccagcagatacagcaagaagttcaagcccgagatcgccaccaggcccaaagtgcgggaccaagagggcagaatgaactactactggaccctggtggaacccggcgacaagatcacattcgaggccaccggcaacctggtggtccccagatacgccttcaccatggaaagagacgccggcagcggcatcatcatcagcgacacccccgtgcacgactgcaacaccacctgccagacacccgagggcgccatcaacaccagcctgcccttccagaacgtgcaccccatcaccatcggcaagtgccccaaatacgtgaagtccaccaagctgaggctggccacaggcctgagaaacgtgcccagcatccagagcagaggcctgttcggagccatcgccggcttcatcgaaggcggctggacaggcatggtggacggatggtacggataccaccaccagaacgagcaaggcagcggctacgccgccgacctgaagtccacccagaacgccatcgacaagatcaccaacaaagtgaacagcgtgatcgagaagatgaacacccagttcaccgccgtgggaaaagagttcaaccacctggaaaagcgcatcgagaacctgaacaagaaggtggacgacggcttcctggacatctggacctacaacgccgagctgctcgtgctgctcgagaacgagagaaccctggactaccacgacagcaacgtgaagaacctgtacgagaaagtgcgcaaccagctgaagaacaacgccaaagagatcggcaacggctgcttcgagttctaccacaagtgcgacaacacctgcatggaaagcgtgaagaacggcacctacgactaccccaagtacagcgaggaagccaaactgaaccgcgagaagatcgacggcgtgaagctggaaagcacccggatctaccagatcctggccatctacagcaccgtggccagcagcctggtgctggtggtgagcctgggcgccatcagcttctggatgtgcagcaacggcagcctgcagtgccggatctgcatctgagctcgctttcttgctgtccaatttctattaaaggttcctttgttccctaagtccaactactaaactgggggatattatgaagggccttgagcatctggattctgcctaataaaaaacatttattttcattgcaaaaaaaaaaaaaaaaaaaaaaaaaaaaaaaaaaaaaaaaaaaaaaaaaaaaaaaaaaaaaaaaaaaaaaaaaaaaaaaaaaaaaaaaaaaaaaacgaagagc

SEQ ID NO: 28 - DNA, 2015 bp, Artificial Sequence
  template DNA sequence for A/Guangdong-Maonan/SWL1536/2019 polyA80
gctagcgtaatacgactcactataaggagacccaagctacatttgcttctgacacaactgtgttcactagcaacctcaaacagacaccgccaccatgaaggccatcctggtggtgctgctgtacaccttcaccaccgccaacgccgacacactgtgcatcggctaccacgccaacaacagcaccgacaccgtggacaccgtgctggaaaagaacgtgaccgtgacacacagcgtgaacctgctggaagacaagcacaacggcaagctgtgcaagctgagaggcgtggcacccctgcacctgggcaagtgcaacatcgccggctggatcctgggcaaccccgagtgcgaaagcctgagcaccgccagaagctggagctacatcgtggaaaccagcaacagcgacaacggcacatgctaccccggcgacttcatcaactacgaggaactgcgggaacagctgagcagcgtgagcagcttcgagagattcgagatcttccccaagaccagcagctggcccaaccacgacagcgacaaaggcgtgacagccgcctgcccccacgccggcgccaagagcttctacaagaacctgatctggctggtcaagaagggcaacagctaccccaagctgaaccagacctacatcaacgacaagggcaaagaggtgctggtcctctggggcatccaccaccccccaacaatcgccgcccaagagagcctgtaccagaacgccgacgcctacgtgttcgtgggcaccagcagatacagcaagaagttcaagcccgagatcgccaccaggcccaaagtgcgggaccaagagggcagaatgaactactactggaccctggtggaacccggcgacaagatcacattcgaggccaccggcaacctggtggtccccagatacgccttcaccatggaaagagacgccggcagcggcatcatcatcagcgacacccccgtgcacgactgcaacaccacctgccagacacccgagggcgccatcaacaccagcctgcccttccagaacgtgcaccccatcaccatcggcaagtgccccaaatacgtgaagtccaccaagctgaggctggccacaggcctgagaaacgtgcccagcatccagagcagaggcctgttcggagccatcgccggcttcatcgaaggcggctggacaggcatggtggacggatggtacggataccaccaccagaacgagcaaggcagcggctacgccgccgacctgaagtccacccagaacgccatcgacaagatcaccaacaaagtgaacagcgtgatcgagaagatgaacacccagttcaccgccgtgggaaaagagttcaaccacctggaaaagcgcatcgagaacctgaacaagaaggtggacgacggcttcctggacatctggacctacaacgccgagctgctcgtgctgctcgagaacgagagaaccctggactaccacgacagcaacgtgaagaacctgtacgagaaagtgcgcaaccagctgaagaacaacgccaaagagatcggcaacggctgcttcgagttctaccacaagtgcgacaacacctgcatggaaagcgtgaagaacggcacctacgactaccccaagtacagcgaggaagccaaactgaaccgcgagaagatcgacggcgtgaagctggaaagcacccggatctaccagatcctggccatctacagcaccgtggccagcagcctggtgctggtggtgagcctgggcgccatcagcttctggatgtgcagcaacggcagcctgcagtgccggatctgcatctgagctcgctttcttgctgtccaatttctattaaaggttcctttgttccctaagtccaactactaaactgggggatattatgaagggccttgagcatctggattctgcctaataaaaaacatttattttcattgcaaaaaaaaaaaaaaaaaaaaaaaaaaaaaaaaaaaaaaaaaaaaaaaaaaaaaaaaaaaaaaaaaaaaaaaaaaaaaaaacgaagagc

SEQ ID NO: 29 - DNA, 1995 bp, Artificial Sequence
  template DNA for A/Guangdong-Maonan/SWL1536/2019 polyA60
gctagcgtaatacgactcactataaggagacccaagctacatttgcttctgacacaactgtgttcactagcaacctcaaacagacaccgccaccatgaaggccatcctggtggtgctgctgtacaccttcaccaccgccaacgccgacacactgtgcatcggctaccacgccaacaacagcaccgacaccgtggacaccgtgctggaaaagaacgtgaccgtgacacacagcgtgaacctgctggaagacaagcacaacggcaagctgtgcaagctgagaggcgtggcacccctgcacctgggcaagtgcaacatcgccggctggatcctgggcaaccccgagtgcgaaagcctgagcaccgccagaagctggagctacatcgtggaaaccagcaacagcgacaacggcacatgctaccccggcgacttcatcaactacgaggaactgcgggaacagctgagcagcgtgagcagcttcgagagattcgagatcttccccaagaccagcagctggcccaaccacgacagcgacaaaggcgtgacagccgcctgcccccacgccggcgccaagagcttctacaagaacctgatctggctggtcaagaagggcaacagctaccccaagctgaaccagacctacatcaacgacaagggcaaagaggtgctggtcctctggggcatccaccaccccccaacaatcgccgcccaagagagcctgtaccagaacgccgacgcctacgtgttcgtgggcaccagcagatacagcaagaagttcaagcccgagatcgccaccaggcccaaagtgcgggaccaagagggcagaatgaactactactggaccctggtggaacccggcgacaagatcacattcgaggccaccggcaacctggtggtccccagatacgccttcaccatggaaagagacgccggcagcggcatcatcatcagcgacacccccgtgcacgactgcaacaccacctgccagacacccgagggcgccatcaacaccagcctgcccttccagaacgtgcaccccatcaccatcggcaagtgccccaaatacgtgaagtccaccaagctgaggctggccacaggcctgagaaacgtgcccagcatccagagcagaggcctgttcggagccatcgccggcttcatcgaaggcggctggacaggcatggtggacggatggtacggataccaccaccagaacgagcaaggcagcggctacgccgccgacctgaagtccacccagaacgccatcgacaagatcaccaacaaagtgaacagcgtgatcgagaagatgaacacccagttcaccgccgtgggaaaagagttcaaccacctggaaaagcgcatcgagaacctgaacaagaaggtggacgacggcttcctggacatctggacctacaacgccgagctgctcgtgctgctcgagaacgagagaaccctggactaccacgacagcaacgtgaagaacctgtacgagaaagtgcgcaaccagctgaagaacaacgccaaagagatcggcaacggctgcttcgagttctaccacaagtgcgacaacacctgcatggaaagcgtgaagaacggcacctacgactaccccaagtacagcgaggaagccaaactgaaccgcgagaagatcgacggcgtgaagctggaaagcacccggatctaccagatcctggccatctacagcaccgtggccagcagcctggtgctggtggtgagcctgggcgccatcagcttctggatgtgcagcaacggcagcctgcagtgccggatctgcatctgagctcgctttcttgctgtccaatttctattaaaggttcctttgttccctaagtccaactactaaactgggggatattatgaagggccttgagcatctggattctgcctaataaaaaacatttattttcattgcaaaaaaaaaaaaaaaaaaaaaaaaaaaaaaaaaaaaaaaaaaaaaaaaaaaaaaaaaaaacgaagagc

SEQ ID NO: 30 - DNA, 1975 bp, Artificial Sequence
  template DNA for A/Guangdong-Maonan/SWL1536/2019 polyA40
gctagcgtaatacgactcactataaggagacccaagctacatttgcttctgacacaactgtgttcactagcaacctcaaacagacaccgccaccatgaaggccatcctggtggtgctgctgtacaccttcaccaccgccaacgccgacacactgtgcatcggctaccacgccaacaacagcaccgacaccgtggacaccgtgctggaaaagaacgtgaccgtgacacacagcgtgaacctgctggaagacaagcacaacggcaagctgtgcaagctgagaggcgtggcacccctgcacctgggcaagtgcaacatcgccggctggatcctgggcaaccccgagtgcgaaagcctgagcaccgccagaagctggagctacatcgtggaaaccagcaacagcgacaacggcacatgctaccccggcgacttcatcaactacgaggaactgcgggaacagctgagcagcgtgagcagcttcgagagattcgagatcttccccaagaccagcagctggcccaaccacgacagcgacaaaggcgtgacagccgcctgcccccacgccggcgccaagagcttctacaagaacctgatctggctggtcaagaagggcaacagctaccccaagctgaaccagacctacatcaacgacaagggcaaagaggtgctggtcctctggggcatccaccaccccccaacaatcgccgcccaagagagcctgtaccagaacgccgacgcctacgtgttcgtgggcaccagcagatacagcaagaagttcaagcccgagatcgccaccaggcccaaagtgcgggaccaagagggcagaatgaactactactggaccctggtggaacccggcgacaagatcacattcgaggccaccggcaacctggtggtccccagatacgccttcaccatggaaagagacgccggcagcggcatcatcatcagcgacacccccgtgcacgactgcaacaccacctgccagacacccgagggcgccatcaacaccagcctgcccttccagaacgtgcaccccatcaccatcggcaagtgccccaaatacgtgaagtccaccaagctgaggctggccacaggcctgagaaacgtgcccagcatccagagcagaggcctgttcggagccatcgccggcttcatcgaaggcggctggacaggcatggtggacggatggtacggataccaccaccagaacgagcaaggcagcggctacgccgccgacctgaagtccacccagaacgccatcgacaagatcaccaacaaagtgaacagcgtgatcgagaagatgaacacccagttcaccgccgtgggaaaagagttcaaccacctggaaaagcgcatcgagaacctgaacaagaaggtggacgacggcttcctggacatctggacctacaacgccgagctgctcgtgctgctcgagaacgagagaaccctggactaccacgacagcaacgtgaagaacctgtacgagaaagtgcgcaaccagctgaagaacaacgccaaagagatcggcaacggctgcttcgagttctaccacaagtgcgacaacacctgcatggaaagcgtgaagaacggcacctacgactaccccaagtacagcgaggaagccaaactgaaccgcgagaagatcgacggcgtgaagctggaaagcacccggatctaccagatcctggccatctacagcaccgtggccagcagcctggtgctggtggtgagcctgggcgccatcagcttctggatgtgcagcaacggcagcctgcagtgccggatctgcatctgagctcgctttcttgctgtccaatttctattaaaggttcctttgttccctaagtccaactactaaactgggggatattatgaagggccttgagcatctggattctgcctaataaaaaacatttattttcattgcaaaaaaaaaaaaaaaaaaaaaaaaaaaaaaaaaaaaaaaacgaagagc

SEQ ID NO: 31 - DNA, 1955 bp, Artificial Sequence
  template DNA for A/Guangdong-Maonan/SWL1536/2019 polyA20
gctagcgtaatacgactcactataaggagacccaagctacatttgcttctgacacaactgtgttcactagcaacctcaaacagacaccgccaccatgaaggccatcctggtggtgctgctgtacaccttcaccaccgccaacgccgacacactgtgcatcggctaccacgccaacaacagcaccgacaccgtggacaccgtgctggaaaagaacgtgaccgtgacacacagcgtgaacctgctggaagacaagcacaacggcaagctgtgcaagctgagaggcgtggcacccctgcacctgggcaagtgcaacatcgccggctggatcctgggcaaccccgagtgcgaaagcctgagcaccgccagaagctggagctacatcgtggaaaccagcaacagcgacaacggcacatgctaccccggcgacttcatcaactacgaggaactgcgggaacagctgagcagcgtgagcagcttcgagagattcgagatcttccccaagaccagcagctggcccaaccacgacagcgacaaaggcgtgacagccgcctgcccccacgccggcgccaagagcttctacaagaacctgatctggctggtcaagaagggcaacagctaccccaagctgaaccagacctacatcaacgacaagggcaaagaggtgctggtcctctggggcatccaccaccccccaacaatcgccgcccaagagagcctgtaccagaacgccgacgcctacgtgttcgtgggcaccagcagatacagcaagaagttcaagcccgagatcgccaccaggcccaaagtgcgggaccaagagggcagaatgaactactactggaccctggtggaacccggcgacaagatcacattcgaggccaccggcaacctggtggtccccagatacgccttcaccatggaaagagacgccggcagcggcatcatcatcagcgacacccccgtgcacgactgcaacaccacctgccagacacccgagggcgccatcaacaccagcctgcccttccagaacgtgcaccccatcaccatcggcaagtgccccaaatacgtgaagtccaccaagctgaggctggccacaggcctgagaaacgtgcccagcatccagagcagaggcctgttcggagccatcgccggcttcatcgaaggcggctggacaggcatggtggacggatggtacggataccaccaccagaacgagcaaggcagcggctacgccgccgacctgaagtccacccagaacgccatcgacaagatcaccaacaaagtgaacagcgtgatcgagaagatgaacacccagttcaccgccgtgggaaaagagttcaaccacctggaaaagcgcatcgagaacctgaacaagaaggtggacgacggcttcctggacatctggacctacaacgccgagctgctcgtgctgctcgagaacgagagaaccctggactaccacgacagcaacgtgaagaacctgtacgagaaagtgcgcaaccagctgaagaacaacgccaaagagatcggcaacggctgcttcgagttctaccacaagtgcgacaacacctgcatggaaagcgtgaagaacggcacctacgactaccccaagtacagcgaggaagccaaactgaaccgcgagaagatcgacggcgtgaagctggaaagcacccggatctaccagatcctggccatctacagcaccgtggccagcagcctggtgctggtggtgagcctgggcgccatcagcttctggatgtgcagcaacggcagcctgcagtgccggatctgcatctgagctcgctttcttgctgtccaatttctattaaaggttcctttgttccctaagtccaactactaaactgggggatattatgaagggccttgagcatctggattctgcctaataaaaaacatttattttcattgcaaaaaaaaaaaaaaaaaaaacgaagagc

SEQ ID NO: 32 - DNA, 2099 bp, Artificial Sequence
  template DNA for B/Phuket/3073/2013(Yamagata lineage) polyA110
gctagcgtaatacgactcactataaggagacccaagctacatttgcttctgacacaactgtgttcactagcaacctcaaacagacaccgccaccatgaaggccatcatcgtgctgctgatggtggtcaccagcaacgccgacagaatctgcaccggcatcaccagcagcaacagcccccacgtggtcaagacagccacacagggcgaagtgaacgtgaccggcgtgatccccctgaccaccacacccaccaagagctacttcgccaacctgaagggcaccagaaccagaggcaagctgtgccccgactgcctgaactgcaccgacctggacgtggccctgggcagacccatgtgcgtgggaacaacacccagcgccaaggccagcatcctgcacgaagtgcggcccgtgaccagcggctgcttccccatcatgcacgaccggaccaagatcagacagctgcccaacctgctgcggggctacgagaagatcaggctgagcacccagaacgtgatcgacgccgaaaaagcccccggcggcccctacagactgggcacaagcggcagctgccccaacgccacaagcaagatcggcttcttcgccaccatggcctgggccgtgcccaaggacaactacaagaacgccaccaaccccctgaccgtggaagtgccctacatctgcaccgaaggcgaggaccagatcaccgtgtggggcttccacagcgacaacaagacccagatgaagtccctgtacggcgacagcaacccccagaagttcaccagcagcgccaacggcgtgaccacacactacgtgagccagatcggcgacttccccgaccagacagaagacggcggactgccccagagcggcagaatcgtggtggactacatgatgcagaagcccggcaagaccggcaccatcgtgtaccagagaggcgtcctgctgccacagaaagtgtggtgcgccagcggccggagcaaagtgatcaaaggaagcctgcccctgatcggcgaggccgactgcctgcacgaagaatacggcggcctgaacaagagcaagccctactacacaggcaagcacgccaaagccatcggcaactgccccatctgggtcaagacccccctgaagctggccaacggcaccaagtacagacccccagccaagctgctgaaagagcggggcttcttcggagccatcgccggcttcctggaaggcggctgggagggaatgatcgccggctggcacggctacacaagccacggcgcacacggcgtggcagtggccgccgacctgaagtccacacaagaggccatcaacaagatcaccaagaacctgaacagcctgagcgagctggaagtgaagaacctgcagagactgagcggcgccatggacgagctgcacaacgagatcctggaactggacgagaaggtggacgacctgagagccgacaccatcagcagccagatcgagctggcagtgctgctgagcaacgagggcatcatcaacagcgaggacgagcacctgctggccctggaacggaagctgaagaagatgctgggacccagcgccgtggacatcggcaacggctgcttcgagacaaagcacaagtgcaaccagacctgcctggacagaatcgccgccggaaccttcaacgccggcgagttcagcctgcccaccttcgacagcctgaacatcacagccgccagcctgaacgacgacggcctggacaaccacaccatcctgctgtactacagcaccgccgccagcagcctggccgtgacactgatgctggccatcttcatcgtgtacatggtgagcagagacaacgtgagctgcagcatctgcctgtgagctcgctttcttgctgtccaatttctattaaaggttcctttgttccctaagtccaactactaaactgggggatattatgaagggccttgagcatctggattctgcctaataaaaaacatttattttcattgcaaaaaaaaaaaaaaaaaaaaaaaaaaaaaaaaaaaaaaaaaaaaaaaaaaaaaaaaaaaaaaaaaaaaaaaaaaaaaaaaaaaaaaaaaaaaaaaaaaaaaaaaaaaaaacgaagagc

SEQ ID NO: 33 - DNA, 2084 bp, Artificial Sequence
  template DNA for B/Phuket/3073/2013(Yamagata lineage) polyA95
gctagcgtaatacgactcactataaggagacccaagctacatttgcttctgacacaactgtgttcactagcaacctcaaacagacaccgccaccatgaaggccatcatcgtgctgctgatggtggtcaccagcaacgccgacagaatctgcaccggcatcaccagcagcaacagcccccacgtggtcaagacagccacacagggcgaagtgaacgtgaccggcgtgatccccctgaccaccacacccaccaagagctacttcgccaacctgaagggcaccagaaccagaggcaagctgtgccccgactgcctgaactgcaccgacctggacgtggccctgggcagacccatgtgcgtgggaacaacacccagcgccaaggccagcatcctgcacgaagtgcggcccgtgaccagcggctgcttccccatcatgcacgaccggaccaagatcagacagctgcccaacctgctgcggggctacgagaagatcaggctgagcacccagaacgtgatcgacgccgaaaaagcccccggcggcccctacagactgggcacaagcggcagctgccccaacgccacaagcaagatcggcttcttcgccaccatggcctgggccgtgcccaaggacaactacaagaacgccaccaaccccctgaccgtggaagtgccctacatctgcaccgaaggcgaggaccagatcaccgtgtggggcttccacagcgacaacaagacccagatgaagtccctgtacggcgacagcaacccccagaagttcaccagcagcgccaacggcgtgaccacacactacgtgagccagatcggcgacttccccgaccagacagaagacggcggactgccccagagcggcagaatcgtggtggactacatgatgcagaagcccggcaagaccggcaccatcgtgtaccagagaggcgtcctgctgccacagaaagtgtggtgcgccagcggccggagcaaagtgatcaaaggaagcctgcccctgatcggcgaggccgactgcctgcacgaagaatacggcggcctgaacaagagcaagccctactacacaggcaagcacgccaaagccatcggcaactgccccatctgggtcaagacccccctgaagctggccaacggcaccaagtacagacccccagccaagctgctgaaagagcggggcttcttcggagccatcgccggcttcctggaaggcggctgggagggaatgatcgccggctggcacggctacacaagccacggcgcacacggcgtggcagtggccgccgacctgaagtccacacaagaggccatcaacaagatcaccaagaacctgaacagcctgagcgagctggaagtgaagaacctgcagagactgagcggcgccatggacgagctgcacaacgagatcctggaactggacgagaaggtggacgacctgagagccgacaccatcagcagccagatcgagctggcagtgctgctgagcaacgagggcatcatcaacagcgaggacgagcacctgctggccctggaacggaagctgaagaagatgctgggacccagcgccgtggacatcggcaacggctgcttcgagacaaagcacaagtgcaaccagacctgcctggacagaatcgccgccggaaccttcaacgccggcgagttcagcctgcccaccttcgacagcctgaacatcacagccgccagcctgaacgacgacggcctggacaaccacaccatcctgctgtactacagcaccgccgccagcagcctggccgtgacactgatgctggccatcttcatcgtgtacatggtgagcagagacaacgtgagctgcagcatctgcctgtgagctcgctttcttgctgtccaatttctattaaaggttcctttgttccctaagtccaactactaaactgggggatattatgaagggccttgagcatctggattctgcctaataaaaaacatttattttcattgcaaaaaaaaaaaaaaaaaaaaaaaaaaaaaaaaaaaaaaaaaaaaaaaaaaaaaaaaaaaaaaaaaaaaaaaaaaaaaaaaaaaaaaaaaaaaaaacgaagagc

SEQ ID NO: 34 - DNA, 2069 bp, Artificial Sequence
  template DNA for B/Phuket/3073/2013(Yamagata lineage) polyA80
gctagcgtaatacgactcactataaggagacccaagctacatttgcttctgacacaactgtgttcactagcaacctcaaacagacaccgccaccatgaaggccatcatcgtgctgctgatggtggtcaccagcaacgccgacagaatctgcaccggcatcaccagcagcaacagcccccacgtggtcaagacagccacacagggcgaagtgaacgtgaccggcgtgatccccctgaccaccacacccaccaagagctacttcgccaacctgaagggcaccagaaccagaggcaagctgtgccccgactgcctgaactgcaccgacctggacgtggccctgggcagacccatgtgcgtgggaacaacacccagcgccaaggccagcatcctgcacgaagtgcggcccgtgaccagcggctgcttccccatcatgcacgaccggaccaagatcagacagctgcccaacctgctgcggggctacgagaagatcaggctgagcacccagaacgtgatcgacgccgaaaaagcccccggcggcccctacagactgggcacaagcggcagctgccccaacgccacaagcaagatcggcttcttcgccaccatggcctgggccgtgcccaaggacaactacaagaacgccaccaaccccctgaccgtggaagtgccctacatctgcaccgaaggcgaggaccagatcaccgtgtggggcttccacagcgacaacaagacccagatgaagtccctgtacggcgacagcaacccccagaagttcaccagcagcgccaacggcgtgaccacacactacgtgagccagatcggcgacttccccgaccagacagaagacggcggactgccccagagcggcagaatcgtggtggactacatgatgcagaagcccggcaagaccggcaccatcgtgtaccagagaggcgtcctgctgccacagaaagtgtggtgcgccagcggccggagcaaagtgatcaaaggaagcctgcccctgatcggcgaggccgactgcctgcacgaagaatacggcggcctgaacaagagcaagccctactacacaggcaagcacgccaaagccatcggcaactgccccatctgggtcaagacccccctgaagctggccaacggcaccaagtacagacccccagccaagctgctgaaagagcggggcttcttcggagccatcgccggcttcctggaaggcggctgggagggaatgatcgccggctggcacggctacacaagccacggcgcacacggcgtggcagtggccgccgacctgaagtccacacaagaggccatcaacaagatcaccaagaacctgaacagcctgagcgagctggaagtgaagaacctgcagagactgagcggcgccatggacgagctgcacaacgagatcctggaactggacgagaaggtggacgacctgagagccgacaccatcagcagccagatcgagctggcagtgctgctgagcaacgagggcatcatcaacagcgaggacgagcacctgctggccctggaacggaagctgaagaagatgctgggacccagcgccgtggacatcggcaacggctgcttcgagacaaagcacaagtgcaaccagacctgcctggacagaatcgccgccggaaccttcaacgccggcgagttcagcctgcccaccttcgacagcctgaacatcacagccgccagcctgaacgacgacggcctggacaaccacaccatcctgctgtactacagcaccgccgccagcagcctggccgtgacactgatgctggccatcttcatcgtgtacatggtgagcagagacaacgtgagctgcagcatctgcctgtgagctcgctttcttgctgtccaatttctattaaaggttcctttgttccctaagtccaactactaaactgggggatattatgaagggccttgagcatctggattctgcctaataaaaaacatttattttcattgcaaaaaaaaaaaaaaaaaaaaaaaaaaaaaaaaaaaaaaaaaaaaaaaaaaaaaaaaaaaaaaaaaaaaaaaaaaaaaaaacgaagagc

SEQ ID NO: 35 - DNA, 2049 bp, Artificial Sequence
  template DNA for B/Phuket/3073/2013(Yamagata lineage) polyA60
gctagcgtaatacgactcactataaggagacccaagctacatttgcttctgacacaactgtgttcactagcaacctcaaacagacaccgccaccatgaaggccatcatcgtgctgctgatggtggtcaccagcaacgccgacagaatctgcaccggcatcaccagcagcaacagcccccacgtggtcaagacagccacacagggcgaagtgaacgtgaccggcgtgatccccctgaccaccacacccaccaagagctacttcgccaacctgaagggcaccagaaccagaggcaagctgtgccccgactgcctgaactgcaccgacctggacgtggccctgggcagacccatgtgcgtgggaacaacacccagcgccaaggccagcatcctgcacgaagtgcggcccgtgaccagcggctgcttccccatcatgcacgaccggaccaagatcagacagctgcccaacctgctgcggggctacgagaagatcaggctgagcacccagaacgtgatcgacgccgaaaaagcccccggcggcccctacagactgggcacaagcggcagctgccccaacgccacaagcaagatcggcttcttcgccaccatggcctgggccgtgcccaaggacaactacaagaacgccaccaaccccctgaccgtggaagtgccctacatctgcaccgaaggcgaggaccagatcaccgtgtggggcttccacagcgacaacaagacccagatgaagtccctgtacggcgacagcaacccccagaagttcaccagcagcgccaacggcgtgaccacacactacgtgagccagatcggcgacttccccgaccagacagaagacggcggactgccccagagcggcagaatcgtggtggactacatgatgcagaagcccggcaagaccggcaccatcgtgtaccagagaggcgtcctgctgccacagaaagtgtggtgcgccagcggccggagcaaagtgatcaaaggaagcctgcccctgatcggcgaggccgactgcctgcacgaagaatacggcggcctgaacaagagcaagccctactacacaggcaagcacgccaaagccatcggcaactgccccatctgggtcaagacccccctgaagctggccaacggcaccaagtacagacccccagccaagctgctgaaagagcggggcttcttcggagccatcgccggcttcctggaaggcggctgggagggaatgatcgccggctggcacggctacacaagccacggcgcacacggcgtggcagtggccgccgacctgaagtccacacaagaggccatcaacaagatcaccaagaacctgaacagcctgagcgagctggaagtgaagaacctgcagagactgagcggcgccatggacgagctgcacaacgagatcctggaactggacgagaaggtggacgacctgagagccgacaccatcagcagccagatcgagctggcagtgctgctgagcaacgagggcatcatcaacagcgaggacgagcacctgctggccctggaacggaagctgaagaagatgctgggacccagcgccgtggacatcggcaacggctgcttcgagacaaagcacaagtgcaaccagacctgcctggacagaatcgccgccggaaccttcaacgccggcgagttcagcctgcccaccttcgacagcctgaacatcacagccgccagcctgaacgacgacggcctggacaaccacaccatcctgctgtactacagcaccgccgccagcagcctggccgtgacactgatgctggccatcttcatcgtgtacatggtgagcagagacaacgtgagctgcagcatctgcctgtgagctcgctttcttgctgtccaatttctattaaaggttcctttgttccctaagtccaactactaaactgggggatattatgaagggccttgagcatctggattctgcctaataaaaaacatttattttcattgcaaaaaaaaaaaaaaaaaaaaaaaaaaaaaaaaaaaaaaaaaaaaaaaaaaaaaaaaaaaacgaagagc

SEQ ID NO: 36 - DNA, 2029 bp, Artificial Sequence
  template DNA for B/Phuket/3073/2013(Yamagata lineage) polyA40
gctagcgtaatacgactcactataaggagacccaagctacatttgcttctgacacaactgtgttcactagcaacctcaaacagacaccgccaccatgaaggccatcatcgtgctgctgatggtggtcaccagcaacgccgacagaatctgcaccggcatcaccagcagcaacagcccccacgtggtcaagacagccacacagggcgaagtgaacgtgaccggcgtgatccccctgaccaccacacccaccaagagctacttcgccaacctgaagggcaccagaaccagaggcaagctgtgccccgactgcctgaactgcaccgacctggacgtggccctgggcagacccatgtgcgtgggaacaacacccagcgccaaggccagcatcctgcacgaagtgcggcccgtgaccagcggctgcttccccatcatgcacgaccggaccaagatcagacagctgcccaacctgctgcggggctacgagaagatcaggctgagcacccagaacgtgatcgacgccgaaaaagcccccggcggcccctacagactgggcacaagcggcagctgccccaacgccacaagcaagatcggcttcttcgccaccatggcctgggccgtgcccaaggacaactacaagaacgccaccaaccccctgaccgtggaagtgccctacatctgcaccgaaggcgaggaccagatcaccgtgtggggcttccacagcgacaacaagacccagatgaagtccctgtacggcgacagcaacccccagaagttcaccagcagcgccaacggcgtgaccacacactacgtgagccagatcggcgacttccccgaccagacagaagacggcggactgccccagagcggcagaatcgtggtggactacatgatgcagaagcccggcaagaccggcaccatcgtgtaccagagaggcgtcctgctgccacagaaagtgtggtgcgccagcggccggagcaaagtgatcaaaggaagcctgcccctgatcggcgaggccgactgcctgcacgaagaatacggcggcctgaacaagagcaagccctactacacaggcaagcacgccaaagccatcggcaactgccccatctgggtcaagacccccctgaagctggccaacggcaccaagtacagacccccagccaagctgctgaaagagcggggcttcttcggagccatcgccggcttcctggaaggcggctgggagggaatgatcgccggctggcacggctacacaagccacggcgcacacggcgtggcagtggccgccgacctgaagtccacacaagaggccatcaacaagatcaccaagaacctgaacagcctgagcgagctggaagtgaagaacctgcagagactgagcggcgccatggacgagctgcacaacgagatcctggaactggacgagaaggtggacgacctgagagccgacaccatcagcagccagatcgagctggcagtgctgctgagcaacgagggcatcatcaacagcgaggacgagcacctgctggccctggaacggaagctgaagaagatgctgggacccagcgccgtggacatcggcaacggctgcttcgagacaaagcacaagtgcaaccagacctgcctggacagaatcgccgccggaaccttcaacgccggcgagttcagcctgcccaccttcgacagcctgaacatcacagccgccagcctgaacgacgacggcctggacaaccacaccatcctgctgtactacagcaccgccgccagcagcctggccgtgacactgatgctggccatcttcatcgtgtacatggtgagcagagacaacgtgagctgcagcatctgcctgtgagctcgctttcttgctgtccaatttctattaaaggttcctttgttccctaagtccaactactaaactgggggatattatgaagggccttgagcatctggattctgcctaataaaaaacatttattttcattgcaaaaaaaaaaaaaaaaaaaaaaaaaaaaaaaaaaaaaaaacgaagagc

SEQ ID NO: 37 - DNA, 2009 bp, Artificial Sequence
  template DNA for B/Phuket/3073/2013(Yamagata lineage) polyA20
gctagcgtaatacgactcactataaggagacccaagctacatttgcttctgacacaactgtgttcactagcaacctcaaacagacaccgccaccatgaaggccatcatcgtgctgctgatggtggtcaccagcaacgccgacagaatctgcaccggcatcaccagcagcaacagcccccacgtggtcaagacagccacacagggcgaagtgaacgtgaccggcgtgatccccctgaccaccacacccaccaagagctacttcgccaacctgaagggcaccagaaccagaggcaagctgtgccccgactgcctgaactgcaccgacctggacgtggccctgggcagacccatgtgcgtgggaacaacacccagcgccaaggccagcatcctgcacgaagtgcggcccgtgaccagcggctgcttccccatcatgcacgaccggaccaagatcagacagctgcccaacctgctgcggggctacgagaagatcaggctgagcacccagaacgtgatcgacgccgaaaaagcccccggcggcccctacagactgggcacaagcggcagctgccccaacgccacaagcaagatcggcttcttcgccaccatggcctgggccgtgcccaaggacaactacaagaacgccaccaaccccctgaccgtggaagtgccctacatctgcaccgaaggcgaggaccagatcaccgtgtggggcttccacagcgacaacaagacccagatgaagtccctgtacggcgacagcaacccccagaagttcaccagcagcgccaacggcgtgaccacacactacgtgagccagatcggcgacttccccgaccagacagaagacggcggactgccccagagcggcagaatcgtggtggactacatgatgcagaagcccggcaagaccggcaccatcgtgtaccagagaggcgtcctgctgccacagaaagtgtggtgcgccagcggccggagcaaagtgatcaaaggaagcctgcccctgatcggcgaggccgactgcctgcacgaagaatacggcggcctgaacaagagcaagccctactacacaggcaagcacgccaaagccatcggcaactgccccatctgggtcaagacccccctgaagctggccaacggcaccaagtacagacccccagccaagctgctgaaagagcggggcttcttcggagccatcgccggcttcctggaaggcggctgggagggaatgatcgccggctggcacggctacacaagccacggcgcacacggcgtggcagtggccgccgacctgaagtccacacaagaggccatcaacaagatcaccaagaacctgaacagcctgagcgagctggaagtgaagaacctgcagagactgagcggcgccatggacgagctgcacaacgagatcctggaactggacgagaaggtggacgacctgagagccgacaccatcagcagccagatcgagctggcagtgctgctgagcaacgagggcatcatcaacagcgaggacgagcacctgctggccctggaacggaagctgaagaagatgctgggacccagcgccgtggacatcggcaacggctgcttcgagacaaagcacaagtgcaaccagacctgcctggacagaatcgccgccggaaccttcaacgccggcgagttcagcctgcccaccttcgacagcctgaacatcacagccgccagcctgaacgacgacggcctggacaaccacaccatcctgctgtactacagcaccgccgccagcagcctggccgtgacactgatgctggccatcttcatcgtgtacatggtgagcagagacaacgtgagctgcagcatctgcctgtgagctcgctttcttgctgtccaatttctattaaaggttcctttgttccctaagtccaactactaaactgggggatattatgaagggccttgagcatctggattctgcctaataaaaaacatttattttcattgcaaaaaaaaaaaaaaaaaaaacgaagagc

SEQ ID NO: 38 - RNA, 2013 nt, Artificial Sequence
  A/Guangdong-Maonan/SWL1536/2019 mRNA polyA110
aggagacccaagcuacauuugcuucugacacaacuguguucacuagcaaccucaaacagacaccgccaccaugaaggccauccugguggugcugcuguacaccuucaccaccgccaacgccgacacacugugcaucggcuaccacgccaacaacagcaccgacaccguggacaccgugcuggaaaagaacgugaccgugacacacagcgugaaccugcuggaagacaagcacaacggcaagcugugcaagcugagaggcguggcaccccugcaccugggcaagugcaacaucgccggcuggauccugggcaaccccgagugcgaaagccugagcaccgccagaagcuggagcuacaucguggaaaccagcaacagcgacaacggcacaugcuaccccggcgacuucaucaacuacgaggaacugcgggaacagcugagcagcgugagcagcuucgagagauucgagaucuuccccaagaccagcagcuggcccaaccacgacagcgacaaaggcgugacagccgccugcccccacgccggcgccaagagcuucuacaagaaccugaucuggcuggucaagaagggcaacagcuaccccaagcugaaccagaccuacaucaacgacaagggcaaagaggugcugguccucuggggcauccaccaccccccaacaaucgccgcccaagagagccuguaccagaacgccgacgccuacguguucgugggcaccagcagauacagcaagaaguucaagcccgagaucgccaccaggcccaaagugcgggaccaagagggcagaaugaacuacuacuggacccugguggaacccggcgacaagaucacauucgaggccaccggcaaccuggugguccccagauacgccuucaccauggaaagagacgccggcagcggcaucaucaucagcgacacccccgugcacgacugcaacaccaccugccagacacccgagggcgccaucaacaccagccugcccuuccagaacgugcaccccaucaccaucggcaagugccccaaauacgugaaguccaccaagcugaggcuggccacaggccugagaaacgugcccagcauccagagcagaggccuguucggagccaucgccggcuucaucgaaggcggcuggacaggcaugguggacggaugguacggauaccaccaccagaacgagcaaggcagcggcuacgccgccgaccugaaguccacccagaacgccaucgacaagaucaccaacaaagugaacagcgugaucgagaagaugaacacccaguucaccgccgugggaaaagaguucaaccaccuggaaaagcgcaucgagaaccugaacaagaagguggacgacggcuuccuggacaucuggaccuacaacgccgagcugcucgugcugcucgagaacgagagaacccuggacuaccacgacagcaacgugaagaaccuguacgagaaagugcgcaaccagcugaagaacaacgccaaagagaucggcaacggcugcuucgaguucuaccacaagugcgacaacaccugcauggaaagcgugaagaacggcaccuacgacuaccccaaguacagcgaggaagccaaacugaaccgcgagaagaucgacggcgugaagcuggaaagcacccggaucuaccagauccuggccaucuacagcaccguggccagcagccuggugcugguggugagccugggcgccaucagcuucuggaugugcagcaacggcagccugcagugccggaucugcaucugagcucgcuuucuugcuguccaauuucuauuaaagguuccuuuguucccuaaguccaacuacuaaacugggggauauuaugaagggccuugagcaucuggauucugccuaauaaaaaacauuuauuuucauugcaaaaaaaaaaaaaaaaaaaaaaaaaaaaaaaaaaaaaaaaaaaaaaaaaaaaaaaaaaaaaaaaaaaaaaaaaaaaaaaaaaaaaaaaaaaaaaaaaaaaaaaaaaaaaa

SEQ ID NO: 39 - RNA, 1998 nt, Artificial Sequence
  A/Guangdong-Maonan/SWL1536/2019 mRNA polyA95
aggagacccaagcuacauuugcuucugacacaacuguguucacuagcaaccucaaacagacaccgccaccaugaaggccauccugguggugcugcuguacaccuucaccaccgccaacgccgacacacugugcaucggcuaccacgccaacaacagcaccgacaccguggacaccgugcuggaaaagaacgugaccgugacacacagcgugaaccugcuggaagacaagcacaacggcaagcugugcaagcugagaggcguggcaccccugcaccugggcaagugcaacaucgccggcuggauccugggcaaccccgagugcgaaagccugagcaccgccagaagcuggagcuacaucguggaaaccagcaacagcgacaacggcacaugcuaccccggcgacuucaucaacuacgaggaacugcgggaacagcugagcagcgugagcagcuucgagagauucgagaucuuccccaagaccagcagcuggcccaaccacgacagcgacaaaggcgugacagccgccugcccccacgccggcgccaagagcuucuacaagaaccugaucuggcuggucaagaagggcaacagcuaccccaagcugaaccagaccuacaucaacgacaagggcaaagaggugcugguccucuggggcauccaccaccccccaacaaucgccgcccaagagagccuguaccagaacgccgacgccuacguguucgugggcaccagcagauacagcaagaaguucaagcccgagaucgccaccaggcccaaagugcgggaccaagagggcagaaugaacuacuacuggacccugguggaacccggcgacaagaucacauucgaggccaccggcaaccuggugguccccagauacgccuucaccauggaaagagacgccggcagcggcaucaucaucagcgacacccccgugcacgacugcaacaccaccugccagacacccgagggcgccaucaacaccagccugcccuuccagaacgugcaccccaucaccaucggcaagugccccaaauacgugaaguccaccaagcugaggcuggccacaggccugagaaacgugcccagcauccagagcagaggccuguucggagccaucgccggcuucaucgaaggcggcuggacaggcaugguggacggaugguacggauaccaccaccagaacgagcaaggcagcggcuacgccgccgaccugaaguccacccagaacgccaucgacaagaucaccaacaaagugaacagcgugaucgagaagaugaacacccaguucaccgccgugggaaaagaguucaaccaccuggaaaagcgcaucgagaaccugaacaagaagguggacgacggcuuccuggacaucuggaccuacaacgccgagcugcucgugcugcucgagaacgagagaacccuggacuaccacgacagcaacgugaagaaccuguacgagaaagugcgcaaccagcugaagaacaacgccaaagagaucggcaacggcugcuucgaguucuaccacaagugcgacaacaccugcauggaaagcgugaagaacggcaccuacgacuaccccaaguacagcgaggaagccaaacugaaccgcgagaagaucgacggcgugaagcuggaaagcacccggaucuaccagauccuggccaucuacagcaccguggccagcagccuggugcugguggugagccugggcgccaucagcuucuggaugugcagcaacggcagccugcagugccggaucugcaucugagcucgcuuucuugcuguccaauuucuauuaaagguuccuuuguucccuaaguccaacuacuaaacugggggauauuaugaagggccuugagcaucuggauucugccuaauaaaaaacauuuauuuucauugcaaaaaaaaaaaaaaaaaaaaaaaaaaaaaaaaaaaaaaaaaaaaaaaaaaaaaaaaaaaaaaaaaaaaaaaaaaaaaaaaaaaaaaaaaaaaaaa

SEQ ID NO: 40 - RNA, 1983 nt, Artificial Sequence
  A/Guangdong-Maonan/SWL1536/2019 mRNA polyA80
aggagacccaagcuacauuugcuucugacacaacuguguucacuagcaaccucaaacagacaccgccaccaugaaggccauccugguggugcugcuguacaccuucaccaccgccaacgccgacacacugugcaucggcuaccacgccaacaacagcaccgacaccguggacaccgugcuggaaaagaacgugaccgugacacacagcgugaaccugcuggaagacaagcacaacggcaagcugugcaagcugagaggcguggcaccccugcaccugggcaagugcaacaucgccggcuggauccugggcaaccccgagugcgaaagccugagcaccgccagaagcuggagcuacaucguggaaaccagcaacagcgacaacggcacaugcuaccccggcgacuucaucaacuacgaggaacugcgggaacagcugagcagcgugagcagcuucgagagauucgagaucuuccccaagaccagcagcuggcccaaccacgacagcgacaaaggcgugacagccgccugcccccacgccggcgccaagagcuucuacaagaaccugaucuggcuggucaagaagggcaacagcuaccccaagcugaaccagaccuacaucaacgacaagggcaaagaggugcugguccucuggggcauccaccaccccccaacaaucgccgcccaagagagccuguaccagaacgccgacgccuacguguucgugggcaccagcagauacagcaagaaguucaagcccgagaucgccaccaggcccaaagugcgggaccaagagggcagaaugaacuacuacuggacccugguggaacccggcgacaagaucacauucgaggccaccggcaaccuggugguccccagauacgccuucaccauggaaagagacgccggcagcggcaucaucaucagcgacacccccgugcacgacugcaacaccaccugccagacacccgagggcgccaucaacaccagccugcccuuccagaacgugcaccccaucaccaucggcaagugccccaaauacgugaaguccaccaagcugaggcuggccacaggccugagaaacgugcccagcauccagagcagaggccuguucggagccaucgccggcuucaucgaaggcggcuggacaggcaugguggacggaugguacggauaccaccaccagaacgagcaaggcagcggcuacgccgccgaccugaaguccacccagaacgccaucgacaagaucaccaacaaagugaacagcgugaucgagaagaugaacacccaguucaccgccgugggaaaagaguucaaccaccuggaaaagcgcaucgagaaccugaacaagaagguggacgacggcuuccuggacaucuggaccuacaacgccgagcugcucgugcugcucgagaacgagagaacccuggacuaccacgacagcaacgugaagaaccuguacgagaaagugcgcaaccagcugaagaacaacgccaaagagaucggcaacggcugcuucgaguucuaccacaagugcgacaacaccugcauggaaagcgugaagaacggcaccuacgacuaccccaaguacagcgaggaagccaaacugaaccgcgagaagaucgacggcgugaagcuggaaagcacccggaucuaccagauccuggccaucuacagcaccguggccagcagccuggugcugguggugagccugggcgccaucagcuucuggaugugcagcaacggcagccugcagugccggaucugcaucugagcucgcuuucuugcuguccaauuucuauuaaagguuccuuuguucccuaaguccaacuacuaaacugggggauauuaugaagggccuugagcaucuggauucugccuaauaaaaaacauuuauuuucauugcaaaaaaaaaaaaaaaaaaaaaaaaaaaaaaaaaaaaaaaaaaaaaaaaaaaaaaaaaaaaaaaaaaaaaaaaaaaaaaaa

SEQ ID NO: 41 - RNA, 1963 nt, Artificial Sequence
  A/Guangdong-Maonan/SWL1536/2019 mRNA polyA60
aggagacccaagcuacauuugcuucugacacaacuguguucacuagcaaccucaaacagacaccgccaccaugaaggccauccugguggugcugcuguacaccuucaccaccgccaacgccgacacacugugcaucggcuaccacgccaacaacagcaccgacaccguggacaccgugcuggaaaagaacgugaccgugacacacagcgugaaccugcuggaagacaagcacaacggcaagcugugcaagcugagaggcguggcaccccugcaccugggcaagugcaacaucgccggcuggauccugggcaaccccgagugcgaaagccugagcaccgccagaagcuggagcuacaucguggaaaccagcaacagcgacaacggcacaugcuaccccggcgacuucaucaacuacgaggaacugcgggaacagcugagcagcgugagcagcuucgagagauucgagaucuuccccaagaccagcagcuggcccaaccacgacagcgacaaaggcgugacagccgccugcccccacgccggcgccaagagcuucuacaagaaccugaucuggcuggucaagaagggcaacagcuaccccaagcugaaccagaccuacaucaacgacaagggcaaagaggugcugguccucuggggcauccaccaccccccaacaaucgccgcccaagagagccuguaccagaacgccgacgccuacguguucgugggcaccagcagauacagcaagaaguucaagcccgagaucgccaccaggcccaaagugcgggaccaagagggcagaaugaacuacuacuggacccugguggaacccggcgacaagaucacauucgaggccaccggcaaccuggugguccccagauacgccuucaccauggaaagagacgccggcagcggcaucaucaucagcgacacccccgugcacgacugcaacaccaccugccagacacccgagggcgccaucaacaccagccugcccuuccagaacgugcaccccaucaccaucggcaagugccccaaauacgugaaguccaccaagcugaggcuggccacaggccugagaaacgugcccagcauccagagcagaggccuguucggagccaucgccggcuucaucgaaggcggcuggacaggcaugguggacggaugguacggauaccaccaccagaacgagcaaggcagcggcuacgccgccgaccugaaguccacccagaacgccaucgacaagaucaccaacaaagugaacagcgugaucgagaagaugaacacccaguucaccgccgugggaaaagaguucaaccaccuggaaaagcgcaucgagaaccugaacaagaagguggacgacggcuuccuggacaucuggaccuacaacgccgagcugcucgugcugcucgagaacgagagaacccuggacuaccacgacagcaacgugaagaaccuguacgagaaagugcgcaaccagcugaagaacaacgccaaagagaucggcaacggcugcuucgaguucuaccacaagugcgacaacaccugcauggaaagcgugaagaacggcaccuacgacuaccccaaguacagcgaggaagccaaacugaaccgcgagaagaucgacggcgugaagcuggaaagcacccggaucuaccagauccuggccaucuacagcaccguggccagcagccuggugcugguggugagccugggcgccaucagcuucuggaugugcagcaacggcagccugcagugccggaucugcaucugagcucgcuuucuugcuguccaauuucuauuaaagguuccuuuguucccuaaguccaacuacuaaacugggggauauuaugaagggccuugagcaucuggauucugccuaauaaaaaacauuuauuuucauugcaaaaaaaaaaaaaaaaaaaaaaaaaaaaaaaaaaaaaaaaaaaaaaaaaaaaaaaaaaaa

SEQ ID NO: 42 - RNA, 1943 nt, Artificial Sequence
  A/Guangdong-Maonan/SWL1536/2019 mRNA polyA40
aggagacccaagcuacauuugcuucugacacaacuguguucacuagcaaccucaaacagacaccgccaccaugaaggccauccugguggugcugcuguacaccuucaccaccgccaacgccgacacacugugcaucggcuaccacgccaacaacagcaccgacaccguggacaccgugcuggaaaagaacgugaccgugacacacagcgugaaccugcuggaagacaagcacaacggcaagcugugcaagcugagaggcguggcaccccugcaccugggcaagugcaacaucgccggcuggauccugggcaaccccgagugcgaaagccugagcaccgccagaagcuggagcuacaucguggaaaccagcaacagcgacaacggcacaugcuaccccggcgacuucaucaacuacgaggaacugcgggaacagcugagcagcgugagcagcuucgagagauucgagaucuuccccaagaccagcagcuggcccaaccacgacagcgacaaaggcgugacagccgccugcccccacgccggcgccaagagcuucuacaagaaccugaucuggcuggucaagaagggcaacagcuaccccaagcugaaccagaccuacaucaacgacaagggcaaagaggugcugguccucuggggcauccaccaccccccaacaaucgccgcccaagagagccuguaccagaacgccgacgccuacguguucgugggcaccagcagauacagcaagaaguucaagcccgagaucgccaccaggcccaaagugcgggaccaagagggcagaaugaacuacuacuggacccugguggaacccggcgacaagaucacauucgaggccaccggcaaccuggugguccccagauacgccuucaccauggaaagagacgccggcagcggcaucaucaucagcgacacccccgugcacgacugcaacaccaccugccagacacccgagggcgccaucaacaccagccugcccuuccagaacgugcaccccaucaccaucggcaagugccccaaauacgugaaguccaccaagcugaggcuggccacaggccugagaaacgugcccagcauccagagcagaggccuguucggagccaucgccggcuucaucgaaggcggcuggacaggcaugguggacggaugguacggauaccaccaccagaacgagcaaggcagcggcuacgccgccgaccugaaguccacccagaacgccaucgacaagaucaccaacaaagugaacagcgugaucgagaagaugaacacccaguucaccgccgugggaaaagaguucaaccaccuggaaaagcgcaucgagaaccugaacaagaagguggacgacggcuuccuggacaucuggaccuacaacgccgagcugcucgugcugcucgagaacgagagaacccuggacuaccacgacagcaacgugaagaaccuguacgagaaagugcgcaaccagcugaagaacaacgccaaagagaucggcaacggcugcuucgaguucuaccacaagugcgacaacaccugcauggaaagcgugaagaacggcaccuacgacuaccccaaguacagcgaggaagccaaacugaaccgcgagaagaucgacggcgugaagcuggaaagcacccggaucuaccagauccuggccaucuacagcaccguggccagcagccuggugcugguggugagccugggcgccaucagcuucuggaugugcagcaacggcagccugcagugccggaucugcaucugagcucgcuuucuugcuguccaauuucuauuaaagguuccuuuguucccuaaguccaacuacuaaacugggggauauuaugaagggccuugagcaucuggauucugccuaauaaaaaacauuuauuuucauugcaaaaaaaaaaaaaaaaaaaaaaaaaaaaaaaaaaaaaaaa

SEQ ID NO: 43 - RNA, 1923 nt, Artificial Sequence
  A/Guangdong-Maonan/SWL1536/2019 mRNA polyA20
aggagacccaagcuacauuugcuucugacacaacuguguucacuagcaaccucaaacagacaccgccaccaugaaggccauccugguggugcugcuguacaccuucaccaccgccaacgccgacacacugugcaucggcuaccacgccaacaacagcaccgacaccguggacaccgugcuggaaaagaacgugaccgugacacacagcgugaaccugcuggaagacaagcacaacggcaagcugugcaagcugagaggcguggcaccccugcaccugggcaagugcaacaucgccggcuggauccugggcaaccccgagugcgaaagccugagcaccgccagaagcuggagcuacaucguggaaaccagcaacagcgacaacggcacaugcuaccccggcgacuucaucaacuacgaggaacugcgggaacagcugagcagcgugagcagcuucgagagauucgagaucuuccccaagaccagcagcuggcccaaccacgacagcgacaaaggcgugacagccgccugcccccacgccggcgccaagagcuucuacaagaaccugaucuggcuggucaagaagggcaacagcuaccccaagcugaaccagaccuacaucaacgacaagggcaaagaggugcugguccucuggggcauccaccaccccccaacaaucgccgcccaagagagccuguaccagaacgccgacgccuacguguucgugggcaccagcagauacagcaagaaguucaagcccgagaucgccaccaggcccaaagugcgggaccaagagggcagaaugaacuacuacuggacccugguggaacccggcgacaagaucacauucgaggccaccggcaaccuggugguccccagauacgccuucaccauggaaagagacgccggcagcggcaucaucaucagcgacacccccgugcacgacugcaacaccaccugccagacacccgagggcgccaucaacaccagccugcccuuccagaacgugcaccccaucaccaucggcaagugccccaaauacgugaaguccaccaagcugaggcuggccacaggccugagaaacgugcccagcauccagagcagaggccuguucggagccaucgccggcuucaucgaaggcggcuggacaggcaugguggacggaugguacggauaccaccaccagaacgagcaaggcagcggcuacgccgccgaccugaaguccacccagaacgccaucgacaagaucaccaacaaagugaacagcgugaucgagaagaugaacacccaguucaccgccgugggaaaagaguucaaccaccuggaaaagcgcaucgagaaccugaacaagaagguggacgacggcuuccuggacaucuggaccuacaacgccgagcugcucgugcugcucgagaacgagagaacccuggacuaccacgacagcaacgugaagaaccuguacgagaaagugcgcaaccagcugaagaacaacgccaaagagaucggcaacggcugcuucgaguucuaccacaagugcgacaacaccugcauggaaagcgugaagaacggcaccuacgacuaccccaaguacagcgaggaagccaaacugaaccgcgagaagaucgacggcgugaagcuggaaagcacccggaucuaccagauccuggccaucuacagcaccguggccagcagccuggugcugguggugagccugggcgccaucagcuucuggaugugcagcaacggcagccugcagugccggaucugcaucugagcucgcuuucuugcuguccaauuucuauuaaagguuccuuuguucccuaaguccaacuacuaaacugggggauauuaugaagggccuugagcaucuggauucugccuaauaaaaaacauuuauuuucauugcaaaaaaaaaaaaaaaaaaaa

SEQ ID NO: 44 - RNA, 2067 nt, Artificial Sequence
  B/Phuket/3073/2013(Yamagata lineage) mRNA polyA110
aggagacccaagcuacauuugcuucugacacaacuguguucacuagcaaccucaaacagacaccgccaccaugaaggccaucaucgugcugcugaugguggucaccagcaacgccgacagaaucugcaccggcaucaccagcagcaacagcccccacguggucaagacagccacacagggcgaagugaacgugaccggcgugaucccccugaccaccacacccaccaagagcuacuucgccaaccugaagggcaccagaaccagaggcaagcugugccccgacugccugaacugcaccgaccuggacguggcccugggcagacccaugugcgugggaacaacacccagcgccaaggccagcauccugcacgaagugcggcccgugaccagcggcugcuuccccaucaugcacgaccggaccaagaucagacagcugcccaaccugcugcggggcuacgagaagaucaggcugagcacccagaacgugaucgacgccgaaaaagcccccggcggccccuacagacugggcacaagcggcagcugccccaacgccacaagcaagaucggcuucuucgccaccauggccugggccgugcccaaggacaacuacaagaacgccaccaacccccugaccguggaagugcccuacaucugcaccgaaggcgaggaccagaucaccguguggggcuuccacagcgacaacaagacccagaugaagucccuguacggcgacagcaacccccagaaguucaccagcagcgccaacggcgugaccacacacuacgugagccagaucggcgacuuccccgaccagacagaagacggcggacugccccagagcggcagaaucgugguggacuacaugaugcagaagcccggcaagaccggcaccaucguguaccagagaggcguccugcugccacagaaaguguggugcgccagcggccggagcaaagugaucaaaggaagccugccccugaucggcgaggccgacugccugcacgaagaauacggcggccugaacaagagcaagcccuacuacacaggcaagcacgccaaagccaucggcaacugccccaucugggucaagaccccccugaagcuggccaacggcaccaaguacagacccccagccaagcugcugaaagagcggggcuucuucggagccaucgccggcuuccuggaaggcggcugggagggaaugaucgccggcuggcacggcuacacaagccacggcgcacacggcguggcaguggccgccgaccugaaguccacacaagaggccaucaacaagaucaccaagaaccugaacagccugagcgagcuggaagugaagaaccugcagagacugagcggcgccauggacgagcugcacaacgagauccuggaacuggacgagaagguggacgaccugagagccgacaccaucagcagccagaucgagcuggcagugcugcugagcaacgagggcaucaucaacagcgaggacgagcaccugcuggcccuggaacggaagcugaagaagaugcugggacccagcgccguggacaucggcaacggcugcuucgagacaaagcacaagugcaaccagaccugccuggacagaaucgccgccggaaccuucaacgccggcgaguucagccugcccaccuucgacagccugaacaucacagccgccagccugaacgacgacggccuggacaaccacaccauccugcuguacuacagcaccgccgccagcagccuggccgugacacugaugcuggccaucuucaucguguacauggugagcagagacaacgugagcugcagcaucugccugugagcucgcuuucuugcuguccaauuucuauuaaagguuccuuuguucccuaaguccaacuacuaaacugggggauauuaugaagggccuugagcaucuggauucugccuaauaaaaaacauuuauuuucauugcaaaaaaaaaaaaaaaaaaaaaaaaaaaaaaaaaaaaaaaaaaaaaaaaaaaaaaaaaaaaaaaaaaaaaaaaaaaaaaaaaaaaaaaaaaaaaaaaaaaaaaaaaaaaaa

SEQ ID NO: 45 - RNA, 2052 nt, Artificial Sequence
  B/Phuket/3073/2013(Yamagata lineage) mRNA polyA95
aggagacccaagcuacauuugcuucugacacaacuguguucacuagcaaccucaaacagacaccgccaccaugaaggccaucaucgugcugcugaugguggucaccagcaacgccgacagaaucugcaccggcaucaccagcagcaacagcccccacguggucaagacagccacacagggcgaagugaacgugaccggcgugaucccccugaccaccacacccaccaagagcuacuucgccaaccugaagggcaccagaaccagaggcaagcugugccccgacugccugaacugcaccgaccuggacguggcccugggcagacccaugugcgugggaacaacacccagcgccaaggccagcauccugcacgaagugcggcccgugaccagcggcugcuuccccaucaugcacgaccggaccaagaucagacagcugcccaaccugcugcggggcuacgagaagaucaggcugagcacccagaacgugaucgacgccgaaaaagcccccggcggccccuacagacugggcacaagcggcagcugccccaacgccacaagcaagaucggcuucuucgccaccauggccugggccgugcccaaggacaacuacaagaacgccaccaacccccugaccguggaagugcccuacaucugcaccgaaggcgaggaccagaucaccguguggggcuuccacagcgacaacaagacccagaugaagucccuguacggcgacagcaacccccagaaguucaccagcagcgccaacggcgugaccacacacuacgugagccagaucggcgacuuccccgaccagacagaagacggcggacugccccagagcggcagaaucgugguggacuacaugaugcagaagcccggcaagaccggcaccaucguguaccagagaggcguccugcugccacagaaaguguggugcgccagcggccggagcaaagugaucaaaggaagccugccccugaucggcgaggccgacugccugcacgaagaauacggcggccugaacaagagcaagcccuacuacacaggcaagcacgccaaagccaucggcaacugccccaucugggucaagaccccccugaagcuggccaacggcaccaaguacagacccccagccaagcugcugaaagagcggggcuucuucggagccaucgccggcuuccuggaaggcggcugggagggaaugaucgccggcuggcacggcuacacaagccacggcgcacacggcguggcaguggccgccgaccugaaguccacacaagaggccaucaacaagaucaccaagaaccugaacagccugagcgagcuggaagugaagaaccugcagagacugagcggcgccauggacgagcugcacaacgagauccuggaacuggacgagaagguggacgaccugagagccgacaccaucagcagccagaucgagcuggcagugcugcugagcaacgagggcaucaucaacagcgaggacgagcaccugcuggcccuggaacggaagcugaagaagaugcugggacccagcgccguggacaucggcaacggcugcuucgagacaaagcacaagugcaaccagaccugccuggacagaaucgccgccggaaccuucaacgccggcgaguucagccugcccaccuucgacagccugaacaucacagccgccagccugaacgacgacggccuggacaaccacaccauccugcuguacuacagcaccgccgccagcagccuggccgugacacugaugcuggccaucuucaucguguacauggugagcagagacaacgugagcugcagcaucugccugugagcucgcuuucuugcuguccaauuucuauuaaagguuccuuuguucccuaaguccaacuacuaaacugggggauauuaugaagggccuugagcaucuggauucugccuaauaaaaaacauuuauuuucauugcaaaaaaaaaaaaaaaaaaaaaaaaaaaaaaaaaaaaaaaaaaaaaaaaaaaaaaaaaaaaaaaaaaaaaaaaaaaaaaaaaaaaaaaaaaaaaaa

SEQ ID NO: 46 - RNA, 2037 nt, Artificial Sequence
  B/Phuket/3073/2013(Yamagata lineage) mRNA polyA80
aggagacccaagcuacauuugcuucugacacaacuguguucacuagcaaccucaaacagacaccgccaccaugaaggccaucaucgugcugcugaugguggucaccagcaacgccgacagaaucugcaccggcaucaccagcagcaacagcccccacguggucaagacagccacacagggcgaagugaacgugaccggcgugaucccccugaccaccacacccaccaagagcuacuucgccaaccugaagggcaccagaaccagaggcaagcugugccccgacugccugaacugcaccgaccuggacguggcccugggcagacccaugugcgugggaacaacacccagcgccaaggccagcauccugcacgaagugcggcccgugaccagcggcugcuuccccaucaugcacgaccggaccaagaucagacagcugcccaaccugcugcggggcuacgagaagaucaggcugagcacccagaacgugaucgacgccgaaaaagcccccggcggccccuacagacugggcacaagcggcagcugccccaacgccacaagcaagaucggcuucuucgccaccauggccugggccgugcccaaggacaacuacaagaacgccaccaacccccugaccguggaagugcccuacaucugcaccgaaggcgaggaccagaucaccguguggggcuuccacagcgacaacaagacccagaugaagucccuguacggcgacagcaacccccagaaguucaccagcagcgccaacggcgugaccacacacuacgugagccagaucggcgacuuccccgaccagacagaagacggcggacugccccagagcggcagaaucgugguggacuacaugaugcagaagcccggcaagaccggcaccaucguguaccagagaggcguccugcugccacagaaaguguggugcgccagcggccggagcaaagugaucaaaggaagccugccccugaucggcgaggccgacugccugcacgaagaauacggcggccugaacaagagcaagcccuacuacacaggcaagcacgccaaagccaucggcaacugccccaucugggucaagaccccccugaagcuggccaacggcaccaaguacagacccccagccaagcugcugaaagagcggggcuucuucggagccaucgccggcuuccuggaaggcggcugggagggaaugaucgccggcuggcacggcuacacaagccacggcgcacacggcguggcaguggccgccgaccugaaguccacacaagaggccaucaacaagaucaccaagaaccugaacagccugagcgagcuggaagugaagaaccugcagagacugagcggcgccauggacgagcugcacaacgagauccuggaacuggacgagaagguggacgaccugagagccgacaccaucagcagccagaucgagcuggcagugcugcugagcaacgagggcaucaucaacagcgaggacgagcaccugcuggcccuggaacggaagcugaagaagaugcugggacccagcgccguggacaucggcaacggcugcuucgagacaaagcacaagugcaaccagaccugccuggacagaaucgccgccggaaccuucaacgccggcgaguucagccugcccaccuucgacagccugaacaucacagccgccagccugaacgacgacggccuggacaaccacaccauccugcuguacuacagcaccgccgccagcagccuggccgugacacugaugcuggccaucuucaucguguacauggugagcagagacaacgugagcugcagcaucugccugugagcucgcuuucuugcuguccaauuucuauuaaagguuccuuuguucccuaaguccaacuacuaaacugggggauauuaugaagggccuugagcaucuggauucugccuaauaaaaaacauuuauuuucauugcaaaaaaaaaaaaaaaaaaaaaaaaaaaaaaaaaaaaaaaaaaaaaaaaaaaaaaaaaaaaaaaaaaaaaaaaaaaaaaaa

SEQ ID NO: 47 - RNA, 2017 nt, Artificial Sequence
  B/Phuket/3073/2013(Yamagata lineage) mRNA polyA60
aggagacccaagcuacauuugcuucugacacaacuguguucacuagcaaccucaaacagacaccgccaccaugaaggccaucaucgugcugcugaugguggucaccagcaacgccgacagaaucugcaccggcaucaccagcagcaacagcccccacguggucaagacagccacacagggcgaagugaacgugaccggcgugaucccccugaccaccacacccaccaagagcuacuucgccaaccugaagggcaccagaaccagaggcaagcugugccccgacugccugaacugcaccgaccuggacguggcccugggcagacccaugugcgugggaacaacacccagcgccaaggccagcauccugcacgaagugcggcccgugaccagcggcugcuuccccaucaugcacgaccggaccaagaucagacagcugcccaaccugcugcggggcuacgagaagaucaggcugagcacccagaacgugaucgacgccgaaaaagcccccggcggccccuacagacugggcacaagcggcagcugccccaacgccacaagcaagaucggcuucuucgccaccauggccugggccgugcccaaggacaacuacaagaacgccaccaacccccugaccguggaagugcccuacaucugcaccgaaggcgaggaccagaucaccguguggggcuuccacagcgacaacaagacccagaugaagucccuguacggcgacagcaacccccagaaguucaccagcagcgccaacggcgugaccacacacuacgugagccagaucggcgacuuccccgaccagacagaagacggcggacugccccagagcggcagaaucgugguggacuacaugaugcagaagcccggcaagaccggcaccaucguguaccagagaggcguccugcugccacagaaaguguggugcgccagcggccggagcaaagugaucaaaggaagccugccccugaucggcgaggccgacugccugcacgaagaauacggcggccugaacaagagcaagcccuacuacacaggcaagcacgccaaagccaucggcaacugccccaucugggucaagaccccccugaagcuggccaacggcaccaaguacagacccccagccaagcugcugaaagagcggggcuucuucggagccaucgccggcuuccuggaaggcggcugggagggaaugaucgccggcuggcacggcuacacaagccacggcgcacacggcguggcaguggccgccgaccugaaguccacacaagaggccaucaacaagaucaccaagaaccugaacagccugagcgagcuggaagugaagaaccugcagagacugagcggcgccauggacgagcugcacaacgagauccuggaacuggacgagaagguggacgaccugagagccgacaccaucagcagccagaucgagcuggcagugcugcugagcaacgagggcaucaucaacagcgaggacgagcaccugcuggcccuggaacggaagcugaagaagaugcugggacccagcgccguggacaucggcaacggcugcuucgagacaaagcacaagugcaaccagaccugccuggacagaaucgccgccggaaccuucaacgccggcgaguucagccugcccaccuucgacagccugaacaucacagccgccagccugaacgacgacggccuggacaaccacaccauccugcuguacuacagcaccgccgccagcagccuggccgugacacugaugcuggccaucuucaucguguacauggugagcagagacaacgugagcugcagcaucugccugugagcucgcuuucuugcuguccaauuucuauuaaagguuccuuuguucccuaaguccaacuacuaaacugggggauauuaugaagggccuugagcaucuggauucugccuaauaaaaaacauuuauuuucauugcaaaaaaaaaaaaaaaaaaaaaaaaaaaaaaaaaaaaaaaaaaaaaaaaaaaaaaaaaaaa

SEQ ID NO: 48 - RNA, 1997 nt, Artificial Sequence
  B/Phuket/3073/2013(Yamagata lineage) mRNA polyA40
aggagacccaagcuacauuugcuucugacacaacuguguucacuagcaaccucaaacagacaccgccaccaugaaggccaucaucgugcugcugaugguggucaccagcaacgccgacagaaucugcaccggcaucaccagcagcaacagcccccacguggucaagacagccacacagggcgaagugaacgugaccggcgugaucccccugaccaccacacccaccaagagcuacuucgccaaccugaagggcaccagaaccagaggcaagcugugccccgacugccugaacugcaccgaccuggacguggcccugggcagacccaugugcgugggaacaacacccagcgccaaggccagcauccugcacgaagugcggcccgugaccagcggcugcuuccccaucaugcacgaccggaccaagaucagacagcugcccaaccugcugcggggcuacgagaagaucaggcugagcacccagaacgugaucgacgccgaaaaagcccccggcggccccuacagacugggcacaagcggcagcugccccaacgccacaagcaagaucggcuucuucgccaccauggccugggccgugcccaaggacaacuacaagaacgccaccaacccccugaccguggaagugcccuacaucugcaccgaaggcgaggaccagaucaccguguggggcuuccacagcgacaacaagacccagaugaagucccuguacggcgacagcaacccccagaaguucaccagcagcgccaacggcgugaccacacacuacgugagccagaucggcgacuuccccgaccagacagaagacggcggacugccccagagcggcagaaucgugguggacuacaugaugcagaagcccggcaagaccggcaccaucguguaccagagaggcguccugcugccacagaaaguguggugcgccagcggccggagcaaagugaucaaaggaagccugccccugaucggcgaggccgacugccugcacgaagaauacggcggccugaacaagagcaagcccuacuacacaggcaagcacgccaaagccaucggcaacugccccaucugggucaagaccccccugaagcuggccaacggcaccaaguacagacccccagccaagcugcugaaagagcggggcuucuucggagccaucgccggcuuccuggaaggcggcugggagggaaugaucgccggcuggcacggcuacacaagccacggcgcacacggcguggcaguggccgccgaccugaaguccacacaagaggccaucaacaagaucaccaagaaccugaacagccugagcgagcuggaagugaagaaccugcagagacugagcggcgccauggacgagcugcacaacgagauccuggaacuggacgagaagguggacgaccugagagccgacaccaucagcagccagaucgagcuggcagugcugcugagcaacgagggcaucaucaacagcgaggacgagcaccugcuggcccuggaacggaagcugaagaagaugcugggacccagcgccguggacaucggcaacggcugcuucgagacaaagcacaagugcaaccagaccugccuggacagaaucgccgccggaaccuucaacgccggcgaguucagccugcccaccuucgacagccugaacaucacagccgccagccugaacgacgacggccuggacaaccacaccauccugcuguacuacagcaccgccgccagcagccuggccgugacacugaugcuggccaucuucaucguguacauggugagcagagacaacgugagcugcagcaucugccugugagcucgcuuucuugcuguccaauuucuauuaaagguuccuuuguucccuaaguccaacuacuaaacugggggauauuaugaagggccuugagcaucuggauucugccuaauaaaaaacauuuauuuucauugcaaaaaaaaaaaaaaaaaaaaaaaaaaaaaaaaaaaaaaaa

SEQ ID NO: 49 - RNA, 1977 nt, Artificial Sequence
  B/Phuket/3073/2013(Yamagata lineage) mRNA polyA20
aggagacccaagcuacauuugcuucugacacaacuguguucacuagcaaccucaaacagacaccgccaccaugaaggccaucaucgugcugcugaugguggucaccagcaacgccgacagaaucugcaccggcaucaccagcagcaacagcccccacguggucaagacagccacacagggcgaagugaacgugaccggcgugaucccccugaccaccacacccaccaagagcuacuucgccaaccugaagggcaccagaaccagaggcaagcugugccccgacugccugaacugcaccgaccuggacguggcccugggcagacccaugugcgugggaacaacacccagcgccaaggccagcauccugcacgaagugcggcccgugaccagcggcugcuuccccaucaugcacgaccggaccaagaucagacagcugcccaaccugcugcggggcuacgagaagaucaggcugagcacccagaacgugaucgacgccgaaaaagcccccggcggccccuacagacugggcacaagcggcagcugccccaacgccacaagcaagaucggcuucuucgccaccauggccugggccgugcccaaggacaacuacaagaacgccaccaacccccugaccguggaagugcccuacaucugcaccgaaggcgaggaccagaucaccguguggggcuuccacagcgacaacaagacccagaugaagucccuguacggcgacagcaacccccagaaguucaccagcagcgccaacggcgugaccacacacuacgugagccagaucggcgacuuccccgaccagacagaagacggcggacugccccagagcggcagaaucgugguggacuacaugaugcagaagcccggcaagaccggcaccaucguguaccagagaggcguccugcugccacagaaaguguggugcgccagcggccggagcaaagugaucaaaggaagccugccccugaucggcgaggccgacugccugcacgaagaauacggcggccugaacaagagcaagcccuacuacacaggcaagcacgccaaagccaucggcaacugccccaucugggucaagaccccccugaagcuggccaacggcaccaaguacagacccccagccaagcugcugaaagagcggggcuucuucggagccaucgccggcuuccuggaaggcggcugggagggaaugaucgccggcuggcacggcuacacaagccacggcgcacacggcguggcaguggccgccgaccugaaguccacacaagaggccaucaacaagaucaccaagaaccugaacagccugagcgagcuggaagugaagaaccugcagagacugagcggcgccauggacgagcugcacaacgagauccuggaacuggacgagaagguggacgaccugagagccgacaccaucagcagccagaucgagcuggcagugcugcugagcaacgagggcaucaucaacagcgaggacgagcaccugcuggcccuggaacggaagcugaagaagaugcugggacccagcgccguggacaucggcaacggcugcuucgagacaaagcacaagugcaaccagaccugccuggacagaaucgccgccggaaccuucaacgccggcgaguucagccugcccaccuucgacagccugaacaucacagccgccagccugaacgacgacggccuggacaaccacaccauccugcuguacuacagcaccgccgccagcagccuggccgugacacugaugcuggccaucuucaucguguacauggugagcagagacaacgugagcugcagcaucugccugugagcucgcuuucuugcuguccaauuucuauuaaagguuccuuuguucccuaaguccaacuacuaaacugggggauauuaugaagggccuugagcaucuggauucugccuaauaaaaaacauuuauuuucauugcaaaaaaaaaaaaaaaaaaaa

SEQ ID NO: 50 - protein, 566 aa, Influenza A virus
MKAILVVLLYTFTTANADTLCIGYHANNSTDTVDTVLEKNVTVTHSVNLLEDKHNGKLCKLRGVAPLHLGKCNIAGWILGNPECESLSTARSWSYIVETSNSDNGTCYPGDFINYEELREQLSSVSSFERFEIFPKTSSWPNHDSDKGVTAACPHAGAKSFYKNLIWLVKKGNSYPKLNQTYINDKGKEVLVLWGIHHPPTIAAQESLYQNADAYVFVGTSRYSKKFKPEIATRPKVRDQEGRMNYYWTLVEPGDKITFEATGNLVVPRYAFTMERDAGSGIIISDTPVHDCNTTCQTPEGAINTSLPFQNVHPITIGKCPKYVKSTKLRLATGLRNVPSIQSRGLFGAIAGFIEGGWTGMVDGWYGYHHQNEQGSGYAADLKSTQNAIDKITNKVNSVIEKMNTQFTAVGKEFNHLEKRIENLNKKVDDGFLDIWTYNAELLVLLENERTLDYHDSNVKNLYEKVRNQLKNNAKEIGNGCFEFYHKCDNTCMESVKNGTYDYPKYSEEAKLNREKIDGVKLESTRIYQILAIYSTVASSLVLVVSLGAISFWMCSNGSLQCRICI

SEQ ID NO: 51 - DNA, 1930 bp, Artificial Sequence
  DNA fragment for A/Astrakhan/3212/2020(H5)HA
gctagcgtaatacgactcactataaggagacccaagctacatttgcttctgacacaactgtgttcactagcaacctcaaacagacaccgccaccatggagaacatagtacttcttcttgcaatagttagccttgttaaaagtgatcagatttgcattggttatcatgcaaacaattcgacagagcaagttgacacgataatggaaaagaacgtcactgttacacatgcccaagacatactggaaaaaacacacaacgggaagctctgtgatctaaatggggtgaagcctctgattttaaaggattgtagtgtagctggatggctcctcggaaacccaatgtgcgacgaattcatcagagtgccggaatggtcctacatagtggagagggctaatccagctaatgacctctgctacccagggagcctcaatgactatgaagaactgaaacacctgttgagcagaataaatcattttgagaagattctgattatccccaagagttcctggccaaaccatgaaacatcactaggggtgagcgcagcttgtccataccagggagcgccctcctttttcagaaatgtggtgtggcttatcaaaaagaacgatgcatacccaacgataaagataagctacaataataccaatcgggaagatctcttgatactgtgggggattcatcattccaacaatgcagaagagcagacaaatctctataaaaacccaaccacctacatttcagttggaacatcaactttaaaccagaggttggtaccaaaaatagctactagatcccaagtaaacgggcaacgtggaagaatggacttcttctggacaattttaaaaccggatgatgcaatccatttcgagagtaatggaaatttcattgctccagaatatgcatacaaaattgtcaagaaaggggactcaacaattatgaaaagtggagtggaatatggccactgcaacaccaaatgtcaaaccccagtaggagcgataaattctagtatgccattccacaacatacatcctctcaccattggggaatgccccaaatacgtgaagtcaaacaagttggtccttgcgactgggctcagaaatagtcctctaagagaaaagagaagaaaaagaggcctgtttggggcgatagcagggtttatagagggaggatggcagggaatggttgatggttggtatgggtaccaccatagcaatgagcaggggagtgggtacgctgcagacaaagaatccacccaaaaggcaatagatggagttaccaataaggtcaactcaatcattgacaaaatgaacactcaatttgaggcagttggaagggagtttaataacttagaaaggaggatagagaatttgaacaagaaaatggaagacggattcctagatgtctggacctataatgctgaacttctagttctcatggaaaacgagaggactctagatttccatgattcaaatgtcaagaacctttacgacaaagtcagactacagcttagggataatgcaaaggagctgggtaacggctgtttcgaattctaccacaaatgcgataatgaatgtatggaaagtgtgagaaatgggacgtatgactaccctcagtattcagaagaagcaagattaaaaagagaagaaataagcggagtgaaattagaatcaataggaacttaccagatactgtcaatttattcaacagcggcgagttccctagcactggcaatcatgatggctggtctatctttatggatgtgctccaatgggtcgttacagtgcagaatttgcatttgagctcgctttcttgctgtccaatttctattaaaggttcctttgttccctaagtccaactactaaactgggggatattatgaagggccttgagcatctggattctgcctaataaaaaacatttattttcattgc

SEQ ID NO: 52 - DNA, 2023 bp, Artificial Sequence
  template DNA for A/Astrakhan/3212/2020(H5)HA
taatacgactcactataaggagacccaagctacatttgcttctgacacaactgtgttcactagcaacctcaaacagacaccgccaccatggagaacatagtacttcttcttgcaatagttagccttgttaaaagtgatcagatttgcattggttatcatgcaaacaattcgacagagcaagttgacacgataatggaaaagaacgtcactgttacacatgcccaagacatactggaaaaaacacacaacgggaagctctgtgatctaaatggggtgaagcctctgattttaaaggattgtagtgtagctggatggctcctcggaaacccaatgtgcgacgaattcatcagagtgccggaatggtcctacatagtggagagggctaatccagctaatgacctctgctacccagggagcctcaatgactatgaagaactgaaacacctgttgagcagaataaatcattttgagaagattctgattatccccaagagttcctggccaaaccatgaaacatcactaggggtgagcgcagcttgtccataccagggagcgccctcctttttcagaaatgtggtgtggcttatcaaaaagaacgatgcatacccaacgataaagataagctacaataataccaatcgggaagatctcttgatactgtgggggattcatcattccaacaatgcagaagagcagacaaatctctataaaaacccaaccacctacatttcagttggaacatcaactttaaaccagaggttggtaccaaaaatagctactagatcccaagtaaacgggcaacgtggaagaatggacttcttctggacaattttaaaaccggatgatgcaatccatttcgagagtaatggaaatttcattgctccagaatatgcatacaaaattgtcaagaaaggggactcaacaattatgaaaagtggagtggaatatggccactgcaacaccaaatgtcaaaccccagtaggagcgataaattctagtatgccattccacaacatacatcctctcaccattggggaatgccccaaatacgtgaagtcaaacaagttggtccttgcgactgggctcagaaatagtcctctaagagaaaagagaagaaaaagaggcctgtttggggcgatagcagggtttatagagggaggatggcagggaatggttgatggttggtatgggtaccaccatagcaatgagcaggggagtgggtacgctgcagacaaagaatccacccaaaaggcaatagatggagttaccaataaggtcaactcaatcattgacaaaatgaacactcaatttgaggcagttggaagggagtttaataacttagaaaggaggatagagaatttgaacaagaaaatggaagacggattcctagatgtctggacctataatgctgaacttctagttctcatggaaaacgagaggactctagatttccatgattcaaatgtcaagaacctttacgacaaagtcagactacagcttagggataatgcaaaggagctgggtaacggctgtttcgaattctaccacaaatgcgataatgaatgtatggaaagtgtgagaaatgggacgtatgactaccctcagtattcagaagaagcaagattaaaaagagaagaaataagcggagtgaaattagaatcaataggaacttaccagatactgtcaatttattcaacagcggcgagttccctagcactggcaatcatgatggctggtctatctttatggatgtgctccaatgggtcgttacagtgcagaatttgcatttgagctcgctttcttgctgtccaatttctattaaaggttcctttgttccctaagtccaactactaaactgggggatattatgaagggccttgagcatctggattctgcctaataaaaaacatttattttcattgcaaaaaaaaaaaaaaaaaaaaaaaaaaaaaaaaaaaaaaaaaaaaaaaaaaaaaaaaaaaaaaaaaaaaaaaaaaaaaaaaaaaaaaaaaaaaaaaaaaaa

SEQ ID NO: 53 - RNA, 2006 nt, Artificial Sequence
  A/Astrakhan/3212/2020(H5)HA mRNA-001
aggagacccaagcuacauuugcuucugacacaacuguguucacuagcaaccucaaacagacaccgccaccauggagaacauaguacuucuucuugcaauaguuagccuuguuaaaagugaucagauuugcauugguuaucaugcaaacaauucgacagagcaaguugacacgauaauggaaaagaacgucacuguuacacaugcccaagacauacuggaaaaaacacacaacgggaagcucugugaucuaaauggggugaagccucugauuuuaaaggauuguaguguagcuggauggcuccucggaaacccaaugugcgacgaauucaucagagugccggaaugguccuacauaguggagagggcuaauccagcuaaugaccucugcuacccagggagccucaaugacuaugaagaacugaaacaccuguugagcagaauaaaucauuuugagaagauucugauuauccccaagaguuccuggccaaaccaugaaacaucacuaggggugagcgcagcuuguccauaccagggagcgcccuccuuuuucagaaaugugguguggcuuaucaaaaagaacgaugcauacccaacgauaaagauaagcuacaauaauaccaaucgggaagaucucuugauacugugggggauucaucauuccaacaaugcagaagagcagacaaaucucuauaaaaacccaaccaccuacauuucaguuggaacaucaacuuuaaaccagagguugguaccaaaaauagcuacuagaucccaaguaaacgggcaacguggaagaauggacuucuucuggacaauuuuaaaaccggaugaugcaauccauuucgagaguaauggaaauuucauugcuccagaauaugcauacaaaauugucaagaaaggggacucaacaauuaugaaaaguggaguggaauauggccacugcaacaccaaaugucaaaccccaguaggagcgauaaauucuaguaugccauuccacaacauacauccucucaccauuggggaaugccccaaauacgugaagucaaacaaguugguccuugcgacugggcucagaaauaguccucuaagagaaaagagaagaaaaagaggccuguuuggggcgauagcaggguuuauagagggaggauggcagggaaugguugaugguugguauggguaccaccauagcaaugagcaggggaguggguacgcugcagacaaagaauccacccaaaaggcaauagauggaguuaccaauaaggucaacucaaucauugacaaaaugaacacucaauuugaggcaguuggaagggaguuuaauaacuuagaaaggaggauagagaauuugaacaagaaaauggaagacggauuccuagaugucuggaccuauaaugcugaacuucuaguucucauggaaaacgagaggacucuagauuuccaugauucaaaugucaagaaccuuuacgacaaagucagacuacagcuuagggauaaugcaaaggagcuggguaacggcuguuucgaauucuaccacaaaugcgauaaugaauguauggaaagugugagaaaugggacguaugacuacccucaguauucagaagaagcaagauuaaaaagagaagaaauaagcggagugaaauuagaaucaauaggaacuuaccagauacugucaauuuauucaacagcggcgaguucccuagcacuggcaaucaugauggcuggucuaucuuuauggaugugcuccaaugggucguuacagugcagaauuugcauuugagcucgcuuucuugcuguccaauuucuauuaaagguuccuuuguucccuaaguccaacuacuaaacugggggauauuaugaagggccuugagcaucuggauucugccuaauaaaaaacauuuauuuucauugcaaaaaaaaaaaaaaaaaaaaaaaaaaaaaaaaaaaaaaaaaaaaaaaaaaaaaaaaaaaaaaaaaaaaaaaaaaaaaaaaaaaaaaaaaaaaaaaaaaaa

SEQ ID NO: 54 - protein, 567 aa, Influenza A virus
MENIVLLLAIVSLVKSDQICIGYHANNSTEQVDTIMEKNVTVTHAQDILEKTHNGKLCDLNGVKPLILKDCSVAGWLLGNPMCDEFIRVPEWSYIVERANPANDLCYPGSLNDYEELKHLLSRINHFEKILIIPKSSWPNHETSLGVSAACPYQGAPSFFRNVVWLIKKNDAYPTIKISYNNTNREDLLILWGIHHSNNAEEQTNLYKNPTTYISVGTSTLNQRLVPKIATRSQVNGQRGRMDFFWTILKPDDAIHFESNGNFIAPEYAYKIVKKGDSTIMKSGVEYGHCNTKCQTPVGAINSSMPFHNIHPLTIGECPKYVKSNKLVLATGLRNSPLREKRRKRGLFGAIAGFIEGGWQGMVDGWYGYHHSNEQGSGYAADKESTQKAIDGVTNKVNSIIDKMNTQFEAVGREFNNLERRIENLNKKMEDGFLDVWTYNAELLVLMENERTLDFHDSNVKNLYDKVRLQLRDNAKELGNGCFEFYHKCDNECMESVRNGTYDYPQYSEEARLKREEISGVKLESIGTYQILSIYSTAASSLALAIMMAGLSLWMCSNGSLQCRICI

SEQ ID NO: 55 - DNA, 1710 bp, Artificial Sequence
  DNA sequence in which the KOZAK sequence and the A/Astrakhan/3212/2020(H5N8) HA gene translated region are linked
gccaccatggagaacatagtacttcttcttgcaatagttagccttgttaaaagtgatcagatttgcattggttatcatgcaaacaattcgacagagcaagttgacacgataatggaaaagaacgtcactgttacacatgcccaagacatactggaaaaaacacacaacgggaagctctgtgatctaaatggggtgaagcctctgattttaaaggattgtagtgtagctggatggctcctcggaaacccaatgtgcgacgaattcatcagagtgccggaatggtcctacatagtggagagggctaatccagctaatgacctctgctacccagggagcctcaatgactatgaagaactgaaacacctgttgagcagaataaatcattttgagaagattctgattatccccaagagttcctggccaaaccatgaaacatcactaggggtgagcgcagcttgtccataccagggagcgccctcctttttcagaaatgtggtgtggcttatcaaaaagaacgatgcatacccaacgataaagataagctacaataataccaatcgggaagatctcttgatactgtgggggattcatcattccaacaatgcagaagagcagacaaatctctataaaaacccaaccacctacatttcagttggaacatcaactttaaaccagaggttggtaccaaaaatagctactagatcccaagtaaacgggcaacgtggaagaatggacttcttctggacaattttaaaaccggatgatgcaatccatttcgagagtaatggaaatttcattgctccagaatatgcatacaaaattgtcaagaaaggggactcaacaattatgaaaagtggagtggaatatggccactgcaacaccaaatgtcaaaccccagtaggagcgataaattctagtatgccattccacaacatacatcctctcaccattggggaatgccccaaatacgtgaagtcaaacaagttggtccttgcgactgggctcagaaatagtcctctaagagaaaagagaagaaaaagaggcctgtttggggcgatagcagggtttatagagggaggatggcagggaatggttgatggttggtatgggtaccaccatagcaatgagcaggggagtgggtacgctgcagacaaagaatccacccaaaaggcaatagatggagttaccaataaggtcaactcaatcattgacaaaatgaacactcaatttgaggcagttggaagggagtttaataacttagaaaggaggatagagaatttgaacaagaaaatggaagacggattcctagatgtctggacctataatgctgaacttctagttctcatggaaaacgagaggactctagatttccatgattcaaatgtcaagaacctttacgacaaagtcagactacagcttagggataatgcaaaggagctgggtaacggctgtttcgaattctaccacaaatgcgataatgaatgtatggaaagtgtgagaaatgggacgtatgactaccctcagtattcagaagaagcaagattaaaaagagaagaaataagcggagtgaaattagaatcaataggaacttaccagatactgtcaatttattcaacagcggcgagttccctagcactggcaatcatgatggctggtctatctttatggatgtgctccaatgggtcgttacagtgcagaatttgcatttaa

SEQ ID NO: 56 - DNA, 1710 bp, Artificial Sequence
  DNA sequence in which the KOZAK sequence and the A/Laos/2122/2020(H5N1)HA gene translated region are linked
gccaccatgaagaaaatagttcttctctttgcaacaatcagccttgtcaaaagcgatcatatttgcattggttaccatgcaaataattcgacagagcaggttgacacaataatggaaaaaaacgttactgttacacaagcccaagacatactggaaaagacacacaacgggaagctctgcgatctaaatggagtgaagcctctgattttaaaagattgtagtgtagcaggatggctcctcggaaatccactgtgtgacgaattcaccaatgtgccagaatggtcttacatagtagagaaggccaatccagccaatgacctctgttacccagggaatttcaatgattatgaagaattgaaacacctattgagcaggataaaccattttgagaaaatacagatcatccccaaaaactcttggtcagatcatgaagcctcattgggggtaagcgccgcgtgttcataccagggaaattcctccttcttcagaaatgtggtgtggcttatcaaaaaggacaatgcatacccaacaataaagaaaggctacaataacaccaatcgagaagatctcctgatactgtgggggatccaccatcctaatgatgaggcagagcagacgaggctctaccaaaacccaactacctatatttccattggaacttcaacattaaaccagaggttggtgccaagaatagccactagacccaaaataaacgggcaaagtggcaggatagatttcttctggacaattttaaaaccgaatgacgcaatccacttcgagagtaatggaaatttcattgctccagaatatgcatacaaaattgtcaagaagggagactccacaatcatgagaagtgaagtaaaatatggtaactgcaacaccaggtgtcagactccaataggagcgataaactctagtatgccattccacaacatacaccctctcactatcggagaatgtcccaaatatgtgaaatcaagcaaattagtccttgcaaccgggctcagaaatagtcctcaaaaagagagaagaagaaaaagaggactgtttggggctatagcaggctttatagagggaggttggcaaggaatggtagatggttggtatgggtaccaccacagtaatgaacaggggagtggttacgctgcagacaaagaatctactcaaaaggcgatagacggggtcaccaataaggtcaattcgatcattgacaaaatgaacactcagtttgaggctgtaggaagggaatttaataacttagagaggagaatagaaaacctaaacaagaaaatggaagatggattcctagatgtctggacttataatgctgaactcctggttctcatggagaatgagagaactctagacttccatgattcaaatgtcaagaacctttatgataaggtccgactacagctcaaggataatgcaaaagaactgggaaacggttgtttcgagttctatcacaaatgtaatgatgaatgtatggaaagtgtaagaaacgggacgtatgactacccgcagtattcagaagaagcaagattaaaaagagaggaaataagtggagtaaaattggaatcaatgggaatctatcaaatactgtcaatttattcaacagtggcgagttccctagtgctggcaatcatgatggctggcctatctttatggatgtgttccaacgggtcgttacagtgcagaatttgcatttag

SEQ ID NO: 57 - DNA, 1701 bp, Artificial Sequence
  DNA sequence for A/Laos/2122/2020(H5N1)HA translated region
atgaagaaaatagttcttctctttgcaacaatcagccttgtcaaaagcgatcatatttgcattggttaccatgcaaataattcgacagagcaggttgacacaataatggaaaaaaacgttactgttacacaagcccaagacatactggaaaagacacacaacgggaagctctgcgatctaaatggagtgaagcctctgattttaaaagattgtagtgtagcaggatggctcctcggaaatccactgtgtgacgaattcaccaatgtgccagaatggtcttacatagtagagaaggccaatccagccaatgacctctgttacccagggaatttcaatgattatgaagaattgaaacacctattgagcaggataaaccattttgagaaaatacagatcatccccaaaaactcttggtcagatcatgaagcctcattgggggtaagcgccgcgtgttcataccagggaaattcctccttcttcagaaatgtggtgtggcttatcaaaaaggacaatgcatacccaacaataaagaaaggctacaataacaccaatcgagaagatctcctgatactgtgggggatccaccatcctaatgatgaggcagagcagacgaggctctaccaaaacccaactacctatatttccattggttcaacattaaaccagaggttggtgccaagaatagccactagacccaaaataaacgggcaaagtggcaggatagatttcttctggacaattttaaaaccgaatgacgcaatccacttcgagagtaatggaaatttcattgctccagaatatgcatacaaaattgtcaagaagggagactccacaatcatgagaagtgaagtaaaatatggtaactgcaacaccaggtgtcagactccaataggagcgataaactctagtatgccattccacaacatacaccctctcactatcggagaatgtcccaaatatgtgaaatcaagcaaattagtccttgcaaccgggctcagaaatagtcctcaaaaagagagaagaagaaaaagaggactgtttggggctatagcaggctttatagagggaggttggcaaggaatggtagatggttggtatgggtaccaccacagtaatgaacaggggagtggttacgctgcagacaaagaatctactcaaaaggcgatagacggggtcaccaataaggtcaattcgatcattgacaaaatgaacactcagtttgaggctgtaggaagggaatttaataacttagagaggagaatagaaaacctaaacaagaaaatggaagatggattcctagatgtctggacttataatgctgaactcctggttctcatggagaatgagagaactctagacttccatgattcaaatgtcaagaacctttatgataaggtccgactacagctcaaggataatgcaaaagaactgggaaacggttgtttcgagttctatcacaaatgtaatgatgaatgtatggaaagtgtaagaaacgggacgtatgactacccgcagtattcagaagaagcaagattaaaaagagaggaaataagtggagtaaaattggaatcaatgggaatctatcaaatactgtcaatttattcaacagtggcgagttccctagtgctggcaatcatgatggctggcctatctttatggatgtgttccaacgggtcgttacagtgcagaatttgcatttag

SEQ ID NO: 58 - protein, 567 aa, Influenza A virus
MKKIVLLFATISLVKSDHICIGYHANNSTEQVDTIMEKNVTVTQAQDILEKTHNGKLCDLNGVKPLILKDCSVAGWLLGNPLCDEFTNVPEWSYIVEKANPANDLCYPGNFNDYEELKHLLSRINHFEKIQIIPKNSWSDHEASLGVSAACSYQGNSSFFRNVVWLIKKDNAYPTIKKGYNNTNREDLLILWGIHHPNDEAEQTRLYQNPTTYISIGTSTLNQRLVPRIATRPKINGQSGRIDFFWTILKPNDAIHFESNGNFIAPEYAYKIVKKGDSTIMRSEVKYGNCNTRCQTPIGAINSSMPFHNIHPLTIGECPKYVKSSKLVLATGLRNSPQKERRRKRGLFGAIAGFIEGGWQGMVDGWYGYHHSNEQGSGYAADKESTQKAIDGVTNKVNSIIDKMNTQFEAVGREFNNLERRIENLNKKMEDGFLDVWTYNAELLVLMENERTLDFHDSNVKNLYDKVRLQLKDNAKELGNGCFEFYHKCNDECMESVRNGTYDYPQYSEEARLKREEISGVKLESMGIYQILSIYSTVASSLVLAIMMAGLSLWMCSNGSLQCRICI